European Patent Specification EP 3 294 877 B1, published June 3, 2026. Title: RAPID CHARACTERIZATION OF TYPE II CAS9 ENDONUCLEASE SYSTEMS, PAM SEQUENCES AND GUIDE RNA ELEMENTS. Applicant: Pioneer Hi-Bred International Inc. Cigan, Andrew Mark Gasiunas, Giedrius Karvelis, Tautvydas Siksnys, Virginijus Young, Joshua K. The sequence listing filed with the application follows.

SEQUENCE LISTING (236 sequences)

SEQ ID NO: 1 - DNA, 20 bp, Artificial Sequence
  synthesized T1 sequence
cgctaaagaggaagaggaca

SEQ ID NO: 2 - DNA, 47 bp, Artificial Sequence
  synthesized GG-821N
  misc_feature (20)..(24): n is a, c, g, or t
tgaccatgattacgaattcnnnnntgtcctcttcctctttagcgagc

SEQ ID NO: 3 - DNA, 44 bp, Artificial Sequence
  synthesized GG-820
aaggatccccgggtaccgagctgctcgctaaagaggaagaggac

SEQ ID NO: 4 - DNA, 22 bp, Artificial Sequence
  synthesized sequence TK-119
gagctcgctaaagaggaagagg

SEQ ID NO: 5 - DNA, 22 bp, Artificial Sequence
  synthesized sequence pUC-dir
gccagggttttcccagtcacga

SEQ ID NO: 6 - DNA, 59 bp, Artificial Sequence
  synthesized sequence JKYS800.1
ctacactctttccctacacgacgctcttccgatctaagtgagctcgctaaagaggaaga

SEQ ID NO: 7 - DNA, 53 bp, Artificial Sequence
  synthesized sequence JKYS803
caagcagaagacggcatacgagctcttccgatctgaattcgagctcggtacct

SEQ ID NO: 8 - DNA, 43 bp, Artificial Sequence
  synthesized sequence Universal Forward
aatgatacggcgaccaccgagatctacactctttccctacacg

SEQ ID NO: 9 - DNA, 18 bp, Artificial Sequence
  synthesized sequence Universal Reverse
caagcagaagacggcata

SEQ ID NO: 10 - DNA, 34 bp, Artificial Sequence
  synthesized sequence Sth1-dir
acgtctcacatgactaagccatactcaattggac

SEQ ID NO: 11 - DNA, 27 bp, Artificial Sequence
  synthesized sequence Sth1-rev
actcgagaccctctcctagtttggcaa

SEQ ID NO: 12 - DNA, 26 bp, Artificial Sequence
  synthesized sequence Sth3-dir
ggggggtctcacatgagtgacttagt

SEQ ID NO: 13 - DNA, 30 bp, Artificial Sequence
  synthesized sequence Sth3-rev
aattactcgagaaaatctagcttaggctta

SEQ ID NO: 14 - DNA, 38 bp, Artificial Sequence
  synthesized sequence Spy-dir
aaggtctcccatggataagaaatactcaataggcttag

SEQ ID NO: 15 - DNA, 32 bp, Artificial Sequence
  synthesized sequence Spy-rev
ttctcgaggtcacctcctagctgactcaaatc

SEQ ID NO: 16 - RNA, 42 nt, Streptococcus thermophilus
cgcuaaagaggaagaggacaguuuuagagcuguguuguuucg

SEQ ID NO: 17 - RNA, 78 nt, Streptococcus thermophilus
gggcgaaacaacacagcgaguuaaaauaaggcuuaguccguacucaacuugaaaagguggcaccgauucgguguuuuu

SEQ ID NO: 18 - RNA, 42 nt, Streptococcus pyogenes
cgcuaaagaggaagaggacaguuuuagagcuaugcuguuuug

SEQ ID NO: 19 - RNA, 78 nt, Streptococcus pyogenes
gggaaacagcauagcaaguuaaaauaaggcuaguccguuaucaacuugaaaaaguggcaccgagucggugcuuuuuuu

SEQ ID NO: 20 - DNA, 31 bp, Artificial Sequence
  synthesized sequence TK-117
cggcattcctgctgaaccgctcttccgatct

SEQ ID NO: 21 - DNA, 30 bp, Artificial Sequence
  synthesized sequence TK-111
gatcggaagagcggttcagcaggaatgccg

SEQ ID NO: 22 - DNA, 56 bp, Artificial Sequence
  synthesized sequence JKYS807.1
ctacactctttccctacacgacgctcttccgatctaaggcggcattcctgctgaac

SEQ ID NO: 23 - DNA, 56 bp, Artificial Sequence
  synthesized sequence JKYS807.2
ctacactctttccctacacgacgctcttccgatctttcccggcattcctgctgaac

SEQ ID NO: 24 - DNA, 56 bp, Artificial Sequence
  synthesized sequence JKYS807.3
ctacactctttccctacacgacgctcttccgatctggaacggcattcctgctgaac

SEQ ID NO: 25 - DNA, 56 bp, Artificial Sequence
  synthesized sequence JKYS807.4
ctacactctttccctacacgacgctcttccgatctccttcggcattcctgctgaac

SEQ ID NO: 26 - RNA, 123 nt, Artificial Sequence
  synthesized sequence Sth3 sgRNA
gggcgcuaaagaggaagaggacaguuuuagagcuguguuguuucgguuaaaacaacacagcgaguuaaaauaaggcuuaguccguacucaacuugaaaagguggcaccgauucgguguuuuuu

SEQ ID NO: 27 - RNA, 105 nt, Artificial Sequence
  synthesized sequence Spy sgRNA
gggcgcuaaagaggaagaggacaguuuuagagcuagaaauagcaaguuaaaauaaggcuaguccguuaucaacuugaaaaaguggcaccgagucggugcuuuuuu

SEQ ID NO: 28 - DNA, 59 bp, Artificial Sequence
  synthesized sequence GG-940-G
  misc_feature (28)..(29): n is a, c, g, or t
  misc_feature (31)..(34): n is a, c, g, or t
gtgcacgccggcgacgttgggtcaactnngnnnntgtcctcttcctctttagcgtttag

SEQ ID NO: 29 - DNA, 59 bp, Artificial Sequence
  synthesized sequence GG-940-C
  misc_feature (28)..(29): n is a, c, g, or t
  misc_feature (31)..(34): n is a, c, g, or t
gtgcacgccggcgacgttgggtcaactnncnnnntgtcctcttcctctttagcgtttag

SEQ ID NO: 30 - DNA, 59 bp, Artificial Sequence
  synthesized sequence GG-940-A
  misc_feature (28)..(29): n is a, c, g, or t
  misc_feature (31)..(34): n is a, c, g, or t
gtgcacgccggcgacgttgggtcaactnnannnntgtcctcttcctctttagcgtttag

SEQ ID NO: 31 - DNA, 59 bp, Artificial Sequence
  synthesized sequence GG-940-T
  misc_feature (28)..(29): n is a, c, g, or t
  misc_feature (31)..(34): n is a, c, g, or t
gtgcacgccggcgacgttgggtcaactnntnnnntgtcctcttcctctttagcgtttag

SEQ ID NO: 32 - DNA, 49 bp, Artificial Sequence
  synthesized sequence JKYS812
caagcagaagacggcatacgagctcttccgatctcggcgacgttgggtc

SEQ ID NO: 33 - RNA, 42 nt, Streptococcus thermophilus
cgcuaaagaggaagaggacaguuuuuguacucucaagauuua

SEQ ID NO: 34 - RNA, 80 nt, Streptococcus thermophilus
ggguaaaucuugcagaagcuacaaagauaaggcuucaugccgaaaucaacacccugucauuuuauggcaggguguuuucg

SEQ ID NO: 35 - protein, 1388 aa, Streptococcus thermophilus
MTKPYSIGLDIGTNSVGWAVITDNYKVPSKKMKVLGNTSKKYIKKNLLGVLLFDSGITAEGRRLKRTARRRYTRRRNRILYLQEIFSTEMATLDDAFFQRLDDSFLVPDDKRDSKYPIFGNLVEEKVYHDEFPTIYHLRKYLADSTKKADLRLVYLALAHMIKYRGHFLIEGEFNSKNNDIQKNFQDFLDTYNAIFESDLSLENSKQLEEIVKDKISKLEKKDRILKLFPGEKNSGIFSEFLKLIVGNQADFRKCFNLDEKASLHFSKESYDEDLETLLGYIGDDYSDVFLKAKKLYDAILLSGFLTVTDNETEAPLSSAMIKRYNEHKEDLALLKEYIRNISLKTYNEVFKDDTKNGYAGYIDGKTNQEDFYVYLKNLLAEFEGADYFLEKIDREDFLRKQRTFDNGSIPYQIHLQEMRAILDKQAKFYPFLAKNKERIEKILTFRIPYYVGPLARGNSDFAWSIRKRNEKITPWNFEDVIDKESSAEAFINRMTSFDLYLPEEKVLPKHSLLYETFNVYNELTKVRFIAESMRDYQFLDSKQKKDIVRLYFKDKRKVTDKDIIEYLHAIYGYDGIELKGIEKQFNSSLSTYHDLLNIINDKEFLDDSSNEAIIEEIIHTLTIFEDREMIKQRLSKFENIFDKSVLKKLSRRHYTGWGKLSAKLINGIRDEKSGNTILDYLIDDGISNRNFMQLIHDDALSFKKKIQKAQIIGDEDKGNIKEVVKSLPGSPAIKKGILQSIKIVDELVKVMGGRKPESIVVEMARENQYTNQGKSNSQQRLKRLEKSLKELGSKILKENIPAKLSKIDNNALQNDRLYLYYLQNGKDMYTGDDLDIDRLSNYDIDHIIPQAFLKDNSIDNKVLVSSASNRGKSDDFPSLEVVKKRKTFWYQLLKSKLISQRKFDNLTKAERGGLLPEDKAGFIQRQLVETRQITKHVARLLDEKFNNKKDENNRAVRTVKIITLKSTLVSQFRKDFELYKVREINDFHHAHDAYLNAVIASALLKKYPKLEPEFVYGDYPKYNSFRERKSATEKVYFYSNIMNIFKKSISLADGRVIERPLIEVNEETGESVWNKESDLATVRRVLSYPQVNVVKKVEEQNHGLDRGKPKGLFNANLSSKPKPNSNENLVGAKEYLDPKKYGGYAGISNSFAVLVKGTIEKGAKKKITNVLEFQGISILDRINYRKDKLNFLLEKGYKDIELIIELPKYSLFELSDGSRRMLASILSTNNKRGEIHKGNQIFLSQKFVKLLYHAKRISNTINENHRKYVENHKKEFEELFYYILEFNENYVGAKKNGKLLNSAFQSWQNHSIDELCSSFIGPTGSERKGLFELTSRGSAADFEFLGVKIPRYRDYTPSSLLKDATLIHQSVTGLYETRIDLAKLGEG

SEQ ID NO: 36 - DNA, 3279 bp, Brevibacillus laterosporus
  misc_feature (1)..(3279): Cas9 single long open-reading-frame
atggcatacacaatgggaatagatgtggggattgcttcgtgtggatgggccattgtagatcttgaaagacaacgaataatagatataggtgttcgaacttttgagaaagcagagaatccgaaaaatggagaggctcttgctgttccaaggagagaagctagatcaagccgtaggagattacggagaaaaaaacatcgcattgaaagattaaagcatatgtttgttcggaatggactggcggttgatattcaacatcttgagcagacgttacgtagtcaaaatgaaatagatgtatggcaattacgagtagatggtttggatcgaatgttaactcaaaaagagtggcttcgtgtattaattcatcttgcacaacgtcgtggttttcaatcaaatcgaaaaacagatggttcaagtgaagatggacaggttcttgtaaatgtaacggagaatgacagattaatggaagagaaagattatagaaccgtagcggaaatgatggtaaaagatgaaaaattttctgaccataagcgaaataaaaatggaaattatcatggagtagtgagcagatcttctttactagttgaaatacatacattatttgaaacccaaagacagcaccataattctttggcatcgaaagatttcgagctggaatatgttaatatttggtctgcacaacggcctgttgcaacaaaagatcaaatagaaaaaatgattggtacatgtactttcttaccgaaagaaaagagagctccaaaggcatcttggcattttcaatattttatgcttttgcaaacgatcaatcatatccgtataacaaatgtacaaggcacgagatcattgaataaagaagaaattgaacaagtggtcaatatggcacttaccaaatcaaaggtatcttaccatgatactagaaagatccttgatttatcagaagaatatcaatttgttggcttggattatggaaaagaggatgaaaaaaagaaagttgaaagtaaggaaacgatcatcaaattagatgattaccataagttaaataagatttttaatgaagtggaattagctaaaggagaaacgtgggaagctgatgattatgatacagtagcgtatgccctcactttctttaaagatgatgaagatattagagattatttgcagaataaatataaagatagtaaaaatcgtcttgttaagaacttggctaataaagaatacacaaatgaattgataggaaaagtgagtacgctatcttttcgtaaagtggggcatttatcattgaaagccttacgaaagatcatcccgtttttggaacaaggtatgacgtatgataaggcgtgccaagcggctggttttgactttcaaggtatatcaaaaaagaagagatctgtcgtcttgccagtcattgaccaaatttccaacccagtagtaaatcgtgctcttactcaaacacgtaaagtaattaatgctctaatcaaaaaatatggttcacctgaaaccatacacattgaaacagcaagagagttatcaaagacatttgatgaacgaaagaatattaccaaggattataaggagaatagagacaagaacgaacatgcaaaaaaacacttatctgaattggggattattaatcctactggtcttgatatagtaaagtacaagttgtggtgtgagcaacaagggcgctgtatgtacagcaatcaacccatctcctttgaaagactgaaagaatcaggttataccgaggtagatcacattattccatacagccgaagtatgaatgatagttataacaatcgcgtattggttatgactagagaaaatcgtgaaaagggtaatcaaactcctttcgaatatatggggaatgatacgcaaagatggtatgagtttgaacagagagtcacaacaaatccacaaataaaaaaggagaaacgacagaacctcttgctaaaaggattcactaatcgtcgggaactagaaatgttagaaagaaacttaaatgatacacgttatataactaagtatctttcacattttattagtacgaatttggaattctctcctagtgataaaaagaaaaaggtagttaatacaagcggtcgtatcacttcccatttaagaagtagatggggattagaaaaaaatcgtgggcaaaatgacctacaccatgcaatggatgcgatcgtcattgctgtcacctcagactcgtttattcaacaggtaacgaattactataaacggaaagaaagaagagagttgaatggggatgataagttccctctaccttggaagttttttagagaagaagtcatagcaagattaagccctaacccaaaagaacaaattgaagcattgcccaaccatttttatagcgaagatgaacttgctgatcttcaaccgatatttgtgtcaagaatgcccaagcgtagtataactggagaggcgcatcaggcacagtttcgtcgagttgtgggtaaaactaaagagggtaaaaatattactgcaaagaaaactgctttagttgatattagctatgataaaaatggtgattttaatatgtatggaagagaaacagatcctgctacttatgaagcaattaaagaaagatatctcgaatttggaggaaatgttaaaaaagcattttcgacggatttacataaaccgaaaaaagatggcaccaaaggtccactgataaaatctgtgagaataatggaaaataaaacattggtacatcccgtaaataaaggaaaaggcgttgtgtataacagctctattgtaaggacagatgtatttcaaagaaaagagaaatattatttactacctgtgtacgtaacagatgtaaccaaggggaaactaccaaataaggtgatcgttgccaaaaagggatatcatgattggattgaggttgatgatagcttcacatttttattcagtctatatccgaatgatttaatattcatcagacaaaatccaaaaaagaaaatatcattaaaaaaacgtattgagagtcattctatttctgatagtaaagaggttcaggaaattcacgcctattataaaggggttgatagttcaactgctgctatagagtttattattcatgatggtagttactatgcaaaaggtgttggtgtccaaaatctagattgttttgaaaaatatcaagttgatattctaggtaattatttcaaagtgaaaggagaaaaacgacttgagttggagacatctgatagtaaccacaaaggcaaagatgtcaattcgattaaatcaactagtcgttaa

SEQ ID NO: 37 - DNA, 36 bp, Brevibacillus laterosporus
  misc_feature (1)..(36): Repeat1
atcatatcatatcgagttttagtaaggaactatagc

SEQ ID NO: 38 - DNA, 36 bp, Brevibacillus laterosporus
  misc_feature (1)..(36): Repeat2
atcatatcatatcgagctttagtaaggaactatagc

SEQ ID NO: 39 - DNA, 36 bp, Brevibacillus laterosporus
  misc_feature (1)..(36): Repeat3
atcatatcatatcgagttttagtaaggaaccatagc

SEQ ID NO: 40 - DNA, 36 bp, Brevibacillus laterosporus; identical to SEQ ID NO: 37
  misc_feature (1)..(36): Repeat4

SEQ ID NO: 41 - DNA, 36 bp, Brevibacillus laterosporus; identical to SEQ ID NO: 37

SEQ ID NO: 42 - DNA, 36 bp, Brevibacillus laterosporus
  misc_feature (1)..(36): Repeat6
atcatatcatatcgagcttcagtaaggaactatagc

SEQ ID NO: 43 - DNA, 36 bp, Brevibacillus laterosporus
  misc_feature (1)..(36): Repeat7
atcatatcatatcaagctttagtaaggaactatagc

SEQ ID NO: 44 - DNA, 36 bp, Brevibacillus laterosporus
  misc_feature (1)..(36): Repeat8
atcatatcatatcgagttttagtaaggaactatagt

SEQ ID NO: 45 - DNA, 29 bp, Artificial Sequence
  synthesized sequence Blat-Cas9-dir
taccatggcatacacaatgggaatagatg

SEQ ID NO: 46 - DNA, 35 bp, Artificial Sequence
  synthesized sequence Blat-Cas9-rev
ttctcgagacgactagttgatttaatcgaattgac

SEQ ID NO: 47 - RNA, 177 nt, Artificial Sequence
  synthesized sequence Blat sgRNA Direct
gggcgcuaaagaggaagaggacagcuauaguuccuuacugaaagguaaguugcuauaguaagggcaacagacccgaggcguuggggaucgccuagcccguuuuuacgggcucuccccauauucaaaauaaugacagacgagcaccuuggagcauuuauuuccgaggugcuuuuuuuu

SEQ ID NO: 48 - RNA, 118 nt, Artificial Sequence
  synthesized sequence Blat sgRNA Reverse
gggcgcuaaagaggaagaggacaaucauaucauaucgaggaaacuugauaugauaugauacuuucauuuuauauccauauaucaucgaagucaaucucauuuaucugucuauuuuaug

SEQ ID NO: 49 - DNA, 68 bp, Artificial Sequence
  synthesized sequence GG-969
gggcgctaaagaggaagaggacagctatagttccttactgaaaggtaagttgctatagtaagggcaac

SEQ ID NO: 50 - DNA, 62 bp, Artificial Sequence
  synthesized sequence GG-839
ctaaaaacgggctaggcgatccccaacgcctcgggtctgttgcccttactatagcaacttac

SEQ ID NO: 51 - DNA, 55 bp, Artificial Sequence
  synthesized sequence TK-149
gatcgcctagcccgtttttacgggctctccccatattcaaaataatgacagacga

SEQ ID NO: 52 - DNA, 62 bp, Artificial Sequence
  synthesized sequence TK-150
aaaaaaaagcacctcggaaataaatgctccaaggtgctcgtctgtcattattttgaatatgg

SEQ ID NO: 53 - DNA, 71 bp, Artificial Sequence
  synthesized sequence GG-840
gggcgctaaagaggaagaggacaatcatatcatatcgaggaaacttgatatgatatgatactttcatttta

SEQ ID NO: 54 - DNA, 75 bp, Artificial Sequence
  synthesized sequence GG-841
cataaaatagacagataaatgagattgacttcgatgatatatggatataaaatgaaagtatcatatcatatcaag

SEQ ID NO: 55 - DNA, 37 bp, Artificial Sequence
  synthesized sequence TK-124
taatacgactcactatagggcgctaaagaggaagagg

SEQ ID NO: 56 - DNA, 26 bp, Artificial Sequence
  synthesized sequence TK-151
aaaaaaaagcacctcggaaataaatg

SEQ ID NO: 57 - DNA, 32 bp, Artificial Sequence
  synthesized sequence TK-126
ataaaatagacagataaatgagattgacttcg

SEQ ID NO: 58 - DNA, 37 bp, Artificial Sequence
  synthesized sequence GG-935
caaattctaaacgctaaagaggaagaggacagtcccg

SEQ ID NO: 59 - DNA, 45 bp, Artificial Sequence
  synthesized sequence GG-936
aattcgggactgtcctcttcctctttagcgtttagaatttgagct

SEQ ID NO: 60 - DNA, 21 bp, Artificial Sequence
  synthesized sequence pUC-EheD
ccgcatcaggcgccattcgcc

SEQ ID NO: 61 - DNA, 22 bp, Artificial Sequence
  synthesized sequence pUC-LguR
gcgaggaagcggaagagcgccc

SEQ ID NO: 62 - DNA, 21 bp, Artificial Sequence
  synthesized sequence Sense DNA Strand of Cleaved Sequencing Template
gaggaagaggaccagtcccgt

SEQ ID NO: 63 - DNA, 11 bp, Artificial Sequence
  synthesized Anti-Sense DNA Strand Sequencing Read
  misc_feature (11)..(11): n is a, c, g, or t
acgggactgtn

SEQ ID NO: 64 - DNA, 21 bp, Artificial Sequence
  synthesized  Anti-Sense DNA Strand of Cleaved Sequencing Template
acgggacctgtcctcttcctc

SEQ ID NO: 65 - DNA, 11 bp, Artificial Sequence
  synthesized  Sense DNA Strand of DNA Sequencing Read
  misc_feature (11)..(11): n is a, c, g, or t
gaggaagaggn

SEQ ID NO: 66 - DNA, 27 bp, Artificial Sequence
  synthesized  Sense DNA Strand of Target and PAM
cgctaaagaggaagaggacagtcccgt

SEQ ID NO: 67 - DNA, 27 bp, Artificial Sequence
  synthesized  Anti-Sense DNA Strand of Target and PAM
acgggactgtcctcttcctctttagcg

SEQ ID NO: 68 - RNA, 118 nt, Brevibacillus laterosporus
  misc_feature (1)..(118): "Direct" tracrRNA region downstream of the anti-repeat
aagggcaacagacccgaggcguuggggaucgccuagcccguuuuuacgggcucuccccauauucaaaauaaugacagacgagcaccuuggagcauuuauuuccgaggugcuuuuuuuu

SEQ ID NO: 69 - RNA, 58 nt, Brevibacillus laterosporus
  misc_feature (1)..(58): "Reverse" tracrRNA region downstream of the anti-repeat
acuuucauuuuauauccauauaucaucgaagucaaucucauuuaucugucuauuuuau

SEQ ID NO: 70 - DNA, 4107 bp, Lactobacillus reuteri
  misc_feature (1)..(4107): Lreu Cas9 Open Reading Frame
atgataaagaaagactataatattggacttgatattggggcaacttcagtcggctttgctggtattgatgaacagtatgacccaattaagttaaagggaaaaacagtagtgggggttaacctatttgaagaagggcaaacagcggcagatcggcgttcctttcgcactacccgtcggcgattgaaccggcgtaaatggcgcttatcattattagaagagttttttgacccatatattacgcctgttgatcccgcattctttgcacgtttgaaggaatcaaatctttcaccaaaggataataacaaaaattttagtagatcattactttttcctgatattacagatcagaaattttatgaagaatatccgacaatttatcatctgcgatatgcattgatgactgaaaataaaaaatttgatcttcgggctatcttcttagcaattcaccatatgatcaagtaccggggaaatttcttaaattccacccctgtagcacattttgatacgagtaagattgattttgcgaatgattttagtaaactaaatcgtctttacttgaatgaagatcctaataatatttttgaaattaatttacaaaatgtaaaagaaataagtgatattttactggatcatagtattaagaagtttgataagcaaaagcaagttgctaagcttttacttacatctcaaaatgataaggaactggataaaagaaataagcagattgctactcagatcagtaaagcaattcttggctataatttttcactaaatgaaattttgaaacttgaagcagtaaataaaagcaaatggaaactaaactttagtagcgccgacattgatgatacgttacccgacttaatttccgaacttgatgaaagtcaagaatcaattttaaatattattttaagtttgtactcacggttgactttaaatggaattgtcccaagtggaatgagtctttccgaatcaatgattgataaatatggtactcataaggaacaccttgatttattaaagaaatatttaaaaacccttcctataaaaaatcggaaagagattgctgaagcctatgccgaatatgttggaaattctttgaagaaaagcggacatatttctcaagaagaattttataaagcagtaaagaagaatcttgataaatccgaaacagctcaaaaaattcttagcttaattagtgaagagaagtttatgcctaagcaacggaccaatcaaaatggggtcattccatatcaacttcaccaaaaggaacttgatcagattattgtaaaccaatctcaatattatccatggttagcagaattaaatccagttacggagcataaagatgcaaagtataaactagatgaattgattgctttccgggtaccgtattatgttggaccgttaattgatcctaaaacaatccctcaaacagaacaaggaaataaaaatgcttcatttgcgtggatggttcgtaaagaaaatggtcaaataacgccatggaattttgataaaaaagtagatagaatttcgtctgcaaataactttattaagcggatgactactaaggatacgtatttaatcggcgaagatgtattacctgctcatagccttatttatgaacgttttaaggtattaaatgaactaaatatgattcgggtaaatggtaaaaaactctctgtttcggttaaacaaaatctttataatgacctatttaaacaacaaaagacaattaataggaagaagttagctaattatctccaagcaaatcttggtatccctgaacgacctcaaattacaggtctctcagatcctgaaaaatttaattcacaattaagctcatatattgatttacaaaaaatactaggaagtgaaattgttgatgatcctaataagcaggatgatttagaaaagattattgaatggtcaactgtttttgaagattcacggatctataaggttaagttacaagaaattggatggttcactgaaaaacaaaagaatgagttagtaagtcatcgctatcaaggctggggacgattatcaaagaaattactagttgagctaaaagataagaatgggagatcaattattgatttgctttggaattcacagcgaacatttatggagattcaaagtcgtccagagtttgctgaacagattactaatgagaaccaagataaattaactgaggataattacgaagacgtactggccgatgcctatacttcaccgcaaaacaaaaaggcaattcgtcaggtaattaaagttgtcgatgatattgttaaggcaactggaaaagcaccgaagtttatttcgttagagtttgctcgctcggatgaacggtcagatcgtgtaaaatcaaggaaaacacatatccaaaaaatttatgaaactaccgctaaagaattactgaaagatgatcagttaattaaagagttaggtagcgtttcagatttatcagatcggttatacttatactttacccagcttggtcgtgatatgtatacaggtaagccaattaatattgatgaaatttcgactatgtatgacattgaccatatccttccgcaggcgtttcttaaggacgattcattagataaccgggtacttgtaagacgacaggataataacgctaaatctgacactgttccggctttgaaatttggaaagatgaaaccattttggaacaaattacaaaagcacggcttgattagtaaacgtaaacttaataacttgcaaactaatcctgaaagtatcgataagtttaaagcagttggttttgtgaaccgtcagttagttgaaacacgccaagttataaaattagctgcaaatattttagcaagccgttatcctgattctaagattattgaagttaaagcaagtttaactcatcaaatgcgtgaatcatttaacctaattaagaatcgggatgttaatgactatcatcatgctgttgatgcgtatttaagtgcatttgtagggcaatacctatataatcgttatcctaaattgcagccatattttgtttatggtcagtttaaaaaatttgataaacaaagtactcggattgggatgaaaactaaccactttaattttttgtatgatcttgagcccgaaggtaaaaatgtaaaaataaagaaaccaactaagattataaacaaggaaactggtgaaattattggtgatcgtgatgaattagttgccaaattgaaccgtgtttataattttaagtacatgttagtttcacaagaagtatatacgcgaagtggtgcattgtttgatcagacaatttacccagctaattcaggtaagaaattaatcccgctgaagcaaaataaaactacagcaatttatggtggatacagtggaagtaaagcagcgtatatgtctatcattaggttacgagataaaaagggtggaacttaccgtatcgttggaatcccagtaagagcagttaataaattaaatcaagcgaagaaaaagagtaatgaaaaatatcttgcagaattaaaggcagtcattgagccacaaattgctaagacaaagaaggatcgaaagactggtcaaagggttcttgtaccacaagaatttgatgtgattatccctgaagttatgtatcgtcagttaatagttgatggtgaccagaaatttacgttgggtggaactattgatagatataatgctgttcaattagttttgaatcaagaaatattgacattccttgagcaacctactaaatataaggacgccgatacaaaattgttggatatatatgatcaaatagtaaatttagtagagaaatattttatgctgtttgatagcaaacgacttgctgcaggtcgagttgcgtttgaaaaattacctactttacaacctgtcgataaaatgccttctaaattaataataattagaagaattattcagggacttcatgacaatgctgctcgaacagatttaaaggcgattaatggaagttcgtcatttggtaggttacaaaaaagaaatggaattatactatcacctaatgcatgcctgatttaccagtcaccaactggcttatttgagagaaaagtttatctaaatactatttcaccattaaaatag

SEQ ID NO: 71 - DNA, 4110 bp, Lactobacillus rossiae
  misc_feature (1)..(4110): Lros Cas9 Open Reading Frame
atggataaatcaaaaccatatggaattggcctagatattggtacaaattctgtcgggttcgtggcgactgatgctgaggggcaccttatccgattgaaaggaaagacggttattggagcgtacctgtttaatgctggaatatcggcagcggaaagacgggggtttcggacgacaagacgtcgattatcgcgggttaaatggcgcctaggacttcttagagaaatatttgagactcattttcaggaaagtatgggagaaaatgaggataatgatttctttttacgtttcaaatactcgaatatttcacctaaagacccacaattttcgacggctaagggtttatttaatgatcgaacggataaggaattttatgatcagtatccgactatttatcatttgcgtcgggctttgatgactgaagaccatcagtttgatattcgggaaatatacatcgcaatgcatcacattgtgaaatatcgtggtcattttttaaaagaaggacgcgccaaagactttaaagttggggatttaagactgctggataatttcaaaatgatgaatgaacaaattgaagaaattaatcctttgtggcagttgaaattaccaactgatgacgcctctattaagtcgataaccgctattttactagacaatactcagagccaaaatgatcgtcaaaaagcagtgacgaaagtaattctggcaacacttgttaaggcgagtgacaaagacattaacgctgcacgtaaacggtttgttggcgaattgagtaaggctatggttggccttaaaacaaaactttgggttcttgcagatgtttcgcagaatggtgattgggaaattaagtatgaaaactacgctgactttgcggaaacgatcggttccggtgaaagtgacaccattcaaagtctttttaacgagattaatgatctatatggggttattacgttggctggcattattcccaaagaagctgagtcattttctgacggaatggtccgcaagtatgaacatcatcgtaaaaatctagaactgttaaaagtttattgtgcggaacaatcagatggtaaacggggacgacagattcgtcagacttatgataaatatattgatggggtagatagcaaacagtttacgcaggaagacttttataaggcattaagcaagttcactgcgaaggatgaagcgactagtgaaaatgccaaattaattgctcaggaaattgcagttggaactttcatgcctaagctgcgaacaaaggctaatggcaccattccacatcagttgcaccaaaaagaattggatgcaattattgaaaatcaaaaaaagtattacccatggcttggtgaagtcaatcccgttgagagtcatcgtcgcgcattgccatacaaattggatgaattagtcagttttaggattccatattatgttggaccaatggttacgccaacaaagggagatccagaaaaaagtaaatttgcctggatggttcgaaaggaaccgggtaccattacgccatggaatttcgatcaaaaagtagaccgatcggcgtctggtgaagcgtttattcaacgaatgaaaacgactgatacatttttaattggcgaagatgtattgccacaacaaagtctgctgtatcagaaatttgaagtactaaatgaattaaacaaaattatgataaacggtaagccaatttgcagagaacagaaacaacggcttttcaaacaactgtttatgcaatataagactgtgacagtgaagaaagttcaacaaaatttaattgcgaatggtgaagagtctgaaaatgtgccaattactggcttgtcagatcctttacggtttaatagttcattcagcacttatatcgattacaaagatattttgggtacagctgctgttaacgataatgcaaagcaaagcgatattgagcagataattgcatggtccacaatttttgaagatgcagccattttccgagagaagttaaatgatattacttggcttaatgacgatcaacgcaataagctcagtcataaacgttatcgcggttggggtcgtcattctcgcaaattgttagctggtcttcgtgacggagaaggccagactatcatcgaacggctatggaacacaaatgacaacttcatgcagattcaaaacgatagtgaaatagcgcgtcaaattaccgaagcaaactcaagcaagatggcaaccgctgagggaacagacgaaattatcgatggcttctacacttcacccgaaaacaaaaaggccctgcgtgaagtaatgaaagttgtgaaggatattcaacgtgcgcatcatggtcaggcacctgcttgggtttatattgaaagtccgcgagagacaccaagacccggtcagcggacagttagtcgagaacaacagttaacagatttgtatgagggtgcagcaaaagaaatcgttgatgatgccgttttaaatgaactaaaggacaaggttaaatccaaggaaaactttacggataaattagttttgtatttcttgcaaaatggacatgatatttatgcgaatgacagtatcaacattgataaccttaatgcatatgatatcgatcatgttttaccgcaaagtttgataaaagatgatagcctagacaatcgggttctcacaacacatgaaagaaatcttaaaaaatctaatcggtttgctacagaactgtttgccgatcaaaggaaaaaatgggaaaaatggcatcgattaggattgatttcgtcacgtaaattaaaacatttaactatgcagcccaattcagtagaaaaatttgcacatggatttattgcacgtcaactcactgaaacgaggcaaataattcatttaacggcgaatgtactttcaaatttatatcaagaaaatgacactaaaatcgttatgattaaggcgggattaaactcggagtttaggcgtacatttgattttccaaagaatcgtagtgtaaatgattaccaccatgcctttgatgcatttttaacggccaaaattggacgttacttattagcgagatatccaaaattagaacccttttttgtttatggaaacttcgttaagaatcctaaagcaatgaagcgattgagtagttttgatttcattgctcagttagctgctaaaactgatgatactagtcatatagatcaacgcagtttaaaacaagttcccgttgttaatgaagaaacaggggaaattgtttgggataaggatattgagcttgctgaactggacaagacgtataactacaaaactatgttagtgaaacgtgctcagactgaaaataatgctcaaatgttcaaacaaacagtttttaaggctcgtgacaatcaaaataaaacgctaattcctgtcaaaaatggattatctactgacgtttatggtggtcattcacaacaggcgatttcttacttatgtatcgtttgggttggacaaaagaaaaaatatcgcgttttgggaattagtaccgcccatgcaggcatattgaacaatttcgaaaaaaactacggccggtttgaagcgaaaaagaaactacaagaaattgtctccaatacactagataatgcggacagaaacgattttaagatagttgctcctaaagttttgtttgaacaagtggttgaggacgataacatgaagtttgggttgggtagtgctagtgactatagaaatgttcaacagttgtttttatcccggaaaaatcagttgctattggctaatatgatgactgaccaaatacacgaccaagatttagtccacctttttgacgaaatagttggtcaaatgaatgcgcattttcccatttttgatcgcggaggctatcgaagttcattgacccaatctcgtgataaatttttgaaattaccttttaaaaagaatgaggatttgatcacgaaacaagaggttattcgaagaattttagatggattacatgctaatgcaaatcgtaaagatcttaaaatcattggtagtaaaggtgattttgggagattgggaacaaagaaaatctacttatcgaaagatgcgaagcttatttacacctcaccaacatgtctttttactcgtactgttccactcagttctttgtaa

SEQ ID NO: 72 - DNA, 4041 bp, Pediococcus pentosaceus
  misc_feature (1)..(4041): Ppen Cas9 Open Reading Frame
atggaaaaagtaccatataatattggtctcgatattgggacgtcatcaattggttttgcagcaaccgataatcttaacaagcctattcgggcaaaaggtaaaaccgttattggagtacgattatttgaagagggtaaaactgcagctgatcgacgtggatttagaacaacacgtcggcgattatcaagaagaaagtggcgtttaaggttacttgatgagattttcgataaagaaatggctaaggtagataataccttttttgctcgtttgaaggagtcgaatctttcaccaaaagatgctaataagaaatatttaggatcattattatttccagaaaagaaggattttaagttttatgaagattatccaacgatatatcatctacgttatgctctaatgcatgaaaaacgtcaatttgatattcgtgaagtttatttagcaatgcatcatattatcaaatatcgtggtaattttttaaattcagccccaatgaattcttttaaaacacaagattttgattttgtggctaaatttgaaaaattaaacgaactctttgaaagtattgatgcggaacatgaaacgaaatttgatattgaaaatatttctaagtttagagatatcatgctaaatcaagatattcgtaagttagaccgaaaaaaacaagccgctaaaattttaatcctagatagtacagataagacggctaaaaagattaataataaaattgcaactgcagtagccaattcagctttaggatataagtttgcgttggatgctattttgaaattagatgtagaagagtctaaagattggtcgattagtttaaacgatgaagaaatcgatagtattttagataacttaactagtgatctggatgcggaacgcatcgaaatcattgagatattgagagatttatacagtcatattgctttaaatgaaattgtacccaacggacaatccttgtctaaatccatgatggataaatacgataagcatcatgcggatttagatgtattgaaaaaagttatttctaatatggacgatcgaaaaaaagctaaatctttaaaaaatatttacaatcagtatgtgggtaaaactaatgataaagttttggataaagatgaattctataaacaaatccaaaagaatttagatgagtctgaagatgctatgaagattgtcaatgaaattgaacttgatcaatttatgccaaaacagcgtacatctcaaaatggagtgattccgcatcaacttcaccaaaaagaattagatgaaatcattgaaaatcaaaagcaatactatccatttttagcagagcctaaccctaacgagaaaagaaaacctcatgctcaatttaaattagatgagttgatagctttcaaaattccttactatgttggtcctttgattacaaaagaagaacaacaagcccaatctggtgctaaatttgcctggatgaagcgtaagcaagatggggtgataactccttggaatttcgatgaaaaagtggatcgaatggcgtcagctaatgaatttattcgccgaatgacgactaaagacacgtatttgttaggtgaagatgtacttccagacgaaagcttaatctatcaaaaatttaaagttttgaatgaattgaataatgtcaaagttaacgataaaaaactgacagtttctgataagcaggatattttcaatgacctgtttaagaaacagaaaactgtttccgtaagtaaacttcaaaagtactttgttacagaaaagcattacttgacagagccaacgatcaaggggttatcagatacgaagaaattttctaatagcttatcaacttatattgattttgaaaaaatatttggaaatgaaattcttgctgatcaaaataagcaaaatgatttagaaaaaattattgagtggtcaactatttttgaagatcgtaaaatttttgaagataaattgcatgagattgaatggttaactgaaaagcagattaaagctgttcggagatatcgtggatggggacggctttctaaaaagctactagtcgatttaagaaataatgaaggtaaaagcattttagatgaactttggcgtaccaatgataactttatgcagattcaagcacgtgaggaatttgctaagtcgattgtcgaagctaaccaaaagttaatgaatcttggtggagctgccagtgttcaaaatactgtggaaagtaccttagaggatgcctatacctctccccaaaataaaaaggctattcgtcaagttattaaagttgttgaagacatagtcaaagcggttggctacgctccagagaaaatcacaattgaatttactcgaggggcagataaaaatcctagacggactcaaaatcgtcaaaagcaaatcatggaagtatataaaaccgcggctaaggaaatcgtagatgcaactttgaagggacaacttgaaaatgaggaaaagttaactgataagttatatttgtatttcacccagttaggtaaagatatttatagtggcgaaacaattaatatcgatcaacttaataattatgatattgaccatattttgccacaagcttttattaaagatgattctctggataatcgagtgttaacaagtcgggatttaaacaacggtaaaagtgatagtgtgcctgtgaagcagtttggtgcaaacatgaaatcattttggatgagactccaagcacatggattaatctcaaaaagaaagcttaataatttaatgacagatccagacagtattggaaaatataccatgcaaggatttgttagaagacagctagttgaaactagccaagttattaagttgactgcaaatatactaggtgccatctatggggaaaatactgatattgtggaaatcccagcgaagctgactcatcaaatgcgggagaagttcaatctgtataaggtgcgtgaggtaaatgattatcatcacgcctttgatgcgtatttaacgacctttgttggtaactatttattcaaacgctatccaaaactacgtccttattttgtatatggcgatttcaaaatgactgataatgccttgaaagggatgcgtagattcaatttcttacatgacttaaaagatgatgaagtattagtagataacgaaactggtgaagttttatgggaaggtcaaaagtctattgaagagttgaagaagatttatggttataagtttatgttaacgactcatgaagcatatacgcaacatggtccaatgtttaagcaaactgtatatagttctgatacgcctggcaaactaattaagataaagaacaataagcctactgaaatatatggtggatatacttcgaatacagatgcttatatggcgattgtaagaataaaagctagaaagggggatacttataaggttgtcggagtacctagaaaagaaggagatgctttaagtcgaatcaagttattagacgaaagtaaataccatgagaacttgaagaatattttagcaattaatttgaataaatctttgaacaagtttgatgtggttctcgataaagttaaatatcggcaggttatttatgacggtacagatcatttaatgttaggtagttcaaaatataaatatagtactaaacaattagtattatcagaccaatctatgaaaattttaagctctactggtgaattctcggacgaggaacttatcaaggtgttcgacgagattatgtacattgttaataagaactttagtttgtatgatacccgaggatttcgtgataagttaaataatgctagggaaaatttcataaaattgcctaataaaacattgttcgaaaagggaaaattaaaacaacatagcaagttagaaatattaaaacaaattttaattggactgcatgcgaatgctggtcgaggtgatttaaaagatattggagttaataattttggagctatggttgttactgctggggtaacgttatcacctgacgctacaattgtttatcaatccccaaccgggctatttgaacgcaaagttaaattgagcgacctttaa

SEQ ID NO: 73 - DNA, 3393 bp, Lactobacillus nodensis
  misc_feature (1)..(3393): Lnod Cas9 Open Reading Frame
atggaaaacaaaattagcttaggattagatattggagttgcttctgttggttttagtgtaattgatgcacaagaaggtaaagtactggagttaggggccagactattcaatagttcagtttccgcggagaatcaaactcgtcgagatatgcgagggtccagaagactaagtaatcgcaagaaacaacgtcgtaaagatgtagctcaactatttaagacttttggattaataaattattttgataaagaaaattattttgataactttcaaaataatttaaattcttatgaattgagagttaaaggattatcagagaaattatcaaaagaagaactggtgaatagtttgtatcatattgtcaaaaggcgtggtatcagttatgacttggcagatgctgacactgatttcgatggttctgattactcatctagtttgaatcagaatcaattggaattacagacgaagactccagctgaaatacaacttactcgcttgaatgtacatggagctgtacgtggaaaagttacgatcaatggcgaggatgaggacactatgcaagtattgttgaatgtgttccccaccaaatcatttgtatctgaagcaaaaaagattattcaaacacaacaacaatattatcctgatattttgacggatatatttgaaactaagtatttagaaattctagaacgtaaaagagaatattttgtcggacctggtagcgaaaaatctagaactgattttggtatctataagaaagatggtagaactttggataatttgttcgaagagttaattggtcatgacaaaatatatcctgatgagttacgtgcgtctggtgcatcttatactgcacaggtttttaatgtcttaaatgatttaaataatttacgtatttctagttatgaaaacgggaaaatttctacggaagataaaataaagattgttgaagatttaagaaacaatatcggcaatgtaattataatgaaaatcattaaaaaggttgccggttgtgaagatgatgatattaaaggctatagattggatagcaaggacaaaccggatattcattcaatggccgtttatcgaaaagttcatcgtgatttattgaaatatgatgtggatattattaagtggccaacggaatttattgatgaattaagtccaatattaactttgaatacggagaacggtgaaattcggaaacaaatggtcaataagttgcaaccaaagtattcatttttaacggatgaacttattcaagttattattaataacaaatctagttttgacgttacttccaataataaatggcatcgtttctcattgaaaacaatgaatgttttgatcgaagaaatgttcagacgaccagttgaacaaatgactcttattcaagaactgggattgattaaagactcaggtaagagatttgaaaattgtaaacttttgccatatagggaaatctcaaaggatatttttaatccggtagcgtccaagtcagttcgtgaggctcttaaaattgttaatgccgtaatgaagaagtatggtcaaattgattatctggttatcgagatgcctcgtgataagaatgaagaagaaatgaagaaacaaattgaaaaattccaaaaggaaaataataagcaaaaagatgaagcaataaatgagtttgttaaaaaaattgggaataagaatgctgttgatgatggactaagacgatatggtggtaaattatatttcaagattagattgtggtatcaacaagatggaattgatttatataatggcaaagtaattgaaccgtttgacttattgaataatattaataaatttgaagtggatcatattattccagaatcaatttcatttgacgacagtattaataacaagacactttgctatgctgatatgaatcaaatcaaaggacaaaagacaccgtttgaatttatgaacgagggacatggccagggctttgcaaaaatgaaggctatggtaaataagaattcaaagttaaaaggtaaacgaaaaaattatttatttgatgaaaatattagtgatattgaaaccagaaaaaggtttatatctcgtaaccttgttgatactcagtattcgtcaagagtggttttgaatagtttgcaagagttctttaaggaaaaagaaaccggaactaaggtgactgtcgtccgaggtaagtttacttctaatttacgcaagcattggcatatcaataagacacgtgatacatttcatcatcacgccatcgatgcatcaataattgccgcgacaccatttttaagaatttggaaaaaagatgccagtttattccccatgcatgtctctgaaaatactgttgatattgaaactggtgagattcttaatgatactgaatttaaaaaagacttttacggattaccgtatagcagttttattgaagaactgaacggtgctgatgaccggattaagttttcgcatcaggttgataggaagatgaatcgtaaggtaagtgatgcgacaatttattcgacacgtaaaggaatgttgaataaagataaagaagaaactgattatgtcttgggaaaaatcaaaaatatttatgatgttagtgagtataacaaattcaaacgaatttacgataaagatccaaataaatttctgttggctcatcatgatccaaaaagctttgatgaacttagaaaaatcatgcaggaatatcctagtaaaattgataaagtaatgactaatggtaaagtaaaatctgtggatatttctccatttgaattgtatcgtcgcaaacatggaatggtacagaaatactctaataaaaataaaggccctgttattaaacaacttaagtatttagacaagaagttgggatctcacattgatattactccgaaggatacattgaatgataggcatgttgtattacagtcactgaagccgtggagaactgatgtgtattacaatagtgtgaccggtgaatatgaaattatgggtattaagtattctgatttgaagttcaatggtggtgagtatggaatcaagatgagcaaatatttggaaataaaagagcgtgaacaggtttcagatgagtctgagtttctgtttactctttataagagagatagaatccaaattataaattgtgaaaatgacgaaattgtagaaatgcttttctggtctagaaataattctaatattgggtatgccgaacttaaaccggtgtataaatataaaactgaggatgaaagttggccggtatacggatatggaaaaaatcaaatcctaaaaagattggtaccaaagaattgtaaaatattgaaagtaaataccgatatactgggcaatccatactatattaaaaaagaatccaaaaacccaaaaaatattcttgattaa

SEQ ID NO: 74 - DNA, 4086 bp, Artificial Sequence
  sequence from Sulfurospirillum sp. SCADC (Sspe)
  misc_feature (1)..(4086): Sspe Cas9 Open Reading Frame
atgacatcgttgatttcactggatttgggtgggaaaaatacgggattttttagttttacagctaaagacgtttcaataatagatacttttcaatcaggaacgattatctatgatgaaagctttgtgctctcacaagtcgcacgacgaggcaaacgacacggtaaacgtaacaacctacgcaacacgctagtcaagcgactttttttgcttcttttacaaaagcattatgggcttagtcttgattttttacccgacgaaattttgggactttttaataaacgaggttacacttatgcaagttttgaaatcaaagaagatgaaaaagaaaatcttgaaagcgatattttaaaagagtttttgaatgacaaactcaattacactatacaaaatgatgacgaagtagaagagtttttaaatcagatagcttcaaatgaagagacgttcaagaactataaaaaggattttgaaaatttatttggagcttcgacgcatcagccaaaaaaacaaattgaacttattgatgagataaaaaaagaccttgaaaaagaagatgccaaagaacttttagatgggttaaaagtcataaaaaaaattatagacgaatttcacaaacaacaaaaccaaggcaatctcccacgggctaagtattttgaagaactttatcttgaaatagaatacaatctaaaaatccaaaaattctttacatgtaaccatcttcacatcaatgacatgcaatatctcatcggcaatctctcaaactatcagctcaaagagctaagacgctactttaacgatgaagctatggcaaaagaagacttttggtcttgcgaaaaactgcatcgcatcacatggcgatttatccaaagttggcacccaaaaagtcctgaagacaaacaaaggcaaaaagagaatcttgcaaaccttaaaaccaaaagtattattgagtttttaaccaccaccaacccactgatgaccattccgccgtatgacgatatgaacaaccgtggagcggtcaaatgccaaacattgcgactcaatgaggagtatttggataagcatctaccacattggagagccatagcacatacgcttgcaagtgagactcaaaaagaaaatcttgagggtgtgaccgtaaaaggctacagtgaagatagcacgcttttacaccgcattttggacacctctagcatcattgacccttatagacttagaagtgatgagatagatagttattgtgatgtattgaccaaagacaatgcttttgcattgaaaaaatttgcaaaagagtactatcaacttgtcaaagaaaaagtacgaacaggtatttggacaaaagacgatgatatgttcaaaaagtgtgaccacaatccaccacacaaaaacaatcaaatccacaatttagtcgcaggaatcttaggcaaacccatcgcaaaagagcggtttgaagcgtttgaaaatgaactttggaatgtaaaatttggcaacaaaaaactctcaagctattgtaaaaacattgaagagtttagaaaatcaaacggcaacctttttaagcagattgtagaattgggtgaagataaagaggtacaaaaatatcaaaaagagttaaacgaatgggtacgaaaaatcggtgagttttttaacatcgaaacgccttatagagcacgctttaacaaccttttttccatggcgcaacttcataccatcatcgataccacacgcagtggttttaacgctacatgtaaatggtgtagctgcgaaaatcaataccgagctagcacaagaatagagatagatgagcaaacaggggaaattactaccaatgccaactgccaacggctcccagccgatacacaaagaccttttagtggcaagattgagcggtacatcgacaaactaggttacgagatagccaaagtcaaagccaaagagttggagggcatcaaagaagatacgatagatttaaaaatcatcttagagcaaaacgcttttgcgtatgaagagtctattcgaaatgccaaaatcaaaaatgccaatgcaaaagctaaaaaagctcttgaagaagcacaaaaaagagggcttaaaaatattgaagacaaaaccaaaagaattaaagattttagcaacagcatttgcccctattgtgggcaaagtttaggcgaagatggcgagatagaccatatcttatcacgaagttacacccttaaaaagtatgataccgttttcaacagcgaaggcaatcttttgtatgttcaccaaaaatgcaatcaagcaaaacttgcaaaaacagattattctttacaagatttaaaaatagatatttctcaaaaatggatagaagaacaaatcgctactatcaaaacctacaaaactttttcagttcttacgcaagaacaacaaaaagcttttaaatatgccctatttttagataactcaaatgaagcttaccaaaaagtaataagttggcttagaaccgaccaaagctcacgagtaaacggtacgcaaaaatatttggctaaaaaaatccaagaaaagctcaaagcgatgtttccagctaaaacatttaactttgagtttatcttagccgatgccaatgatgtgcatgatttgagaattaaagcgtatcaattgccagaaaagccaaaagactctaaacaagaaacctacagtcatactatagatgcggttatgagtttggtcagtgtatgggataaggtattgccaaaaacagaaaaacctacaaaagaagatattttaaaatttgccaatgtcgaaaattggagtgccctcaataatgaatttttaaccaaaggcaaatcagcaaatcaaaaaatagaagagatgatacaagccaatgattttggtcaaaaaaatatgaggcaagtttttagtaagcccatttttaaagatgaatcaataggagaaaggtataagccatttgttcgctatcacaatcaattttacataggctatccgataagcataaaagacggatacgatatgcagcattgtcaagcaatgatttcaaagaacgatatttcaagggtagaggagattcttaaagacacctctttatgcactcttttaaaagaaaagaatggcattaaactttattctattaacaagcaaagtatcaatgaactgtcaaatcagttctttaatttaaactatcaaaacttaaacgatgcacagaagaaaaaatctgaactggcagaatttgtcatcaatcattgtaaatattatgtcaaaaaaacatcggttatcaatgcgccacaatttattgataaagattcgatgaagccgtacccgttttataaagactggcaaaaatttcacgaagcttacaaaaaagagcttgatgctgaaccaaaaaccaaaaaagataacgggaaattagtttatgatatatcaggcatagatgacttctggactgaattttgcaaaaaatattttggtataaaaacaaaagacaatcgaaacaaagcgagaaaggttttttctattgtggcgcttacttcagccccaggaacagtctttagaatcaaacgaaaaacgcctaaaggacacatataccaagcaacggcgattgacaatcaacaaatcagcggagattatgcaaatgttctgttagctggtaactcaaaaacacttgcgttggcaggtcaaaaaccttcatctgacttgaaaaaagagttgagtgtcaaagagtcaaaagatattcgagatataaagcttgagccatcaagatttttcaaagaggggtttgattgtcgtggcattgaagttattgtcaataaaacaagtgcgaccattaaaaatttcccacttacaaaaattgataaaaaaatcaaaaaacttatttttaaaactctctttgaaaaaaaagatggtaaacgacaaaagcaaaaaacatcaatttcattgaaagaaaaaaatacaatgcaagagacactaaaaaaattattaaaagatagtataaaagttactattagagatggtagcatttcgggtattgaaattagcaaaaaaactgttaattttactttgccgttcaaaagtgaaaacttggcaaaactcttagatgactaa

SEQ ID NO: 75 - DNA, 3444 bp, Bifidobacterium thermophilum
  misc_feature (1)..(3444): Bthe Cas9 Open Reading Frame
atgtctgataagacatatcgtatcggtatcgacgttggtttgtactctgttggcttgtctgccattcaggtaaatgatgatgacgatccagtaagaatactgaacgcacagagtgtcatccatgatggcggtgtcgatccgaatgctcagaaaagcgctgatagccgacgtgctcagtctgggattgcccgtcgcacgcgtcgtatgcgccgtaataggaagaaacgtctgaagcgtcttgatcaaattcttgtggaatctggtttccctgtgagcagtgagaatgatcttgaaggatttgaaccgtggcttcttagggcgcaagcggctgatgccttcattgaagatgaggatattcgcaagcgtgcaatttcggtttcatgtcgccatatcgcgcgccatcgtggatggagaaatccttatttggatgttcgaacgctgctggcggttgactcgccttcctcggcattctatgacaagctcgtggagaatgctgctcttgaaatggacggccagatgcctgacagcgatgccacgccggcacagattgtgcgcgatgtgcttgagtacaagcgtggtgaagctgctatccgtcttcgaaagtcaacggctgagaataagaaaaatcgcctcgctttgttccctgagaagatgatgcaggatgactatgcttatgaattgcgtttgattctggcgaagcaagcggttcccaaagatatcgctcgcaagctcattttggcggtgttccaatcgcagtcgccaaaaggttctgcggagaagcgtgttgggaaagatccccttgatccgtctcagcctcgggctttgaaggcttctctggcattccaagaatatcgaatattgaatattcttaccaatctgcgtttgcaggatggtggcgcggagcgtcgtctgtctattgaggaaaagcagaagctctacaagatgctcgtggaagatacgggtcgcgaaaagaagtacgagacatggacagatatcgcatcggccatggagtggaagcgaaattggctcaagggagttgggagtttgacggccgatggcgatgaccgagtcactagtcgccctcctcatatcgatattgtagaaaagctcaacggcattaaggatacgaaattcagaaagagtattttgtcgtggtggaaatctgcgactgatgtcaaccgtgaagcgatgattgccctgctttccaatacagtcgatatcgccaagaaacaggatgacccggatttctcatccgccgtggatttcattgattcgatggatgatagcgatttgcagattctcgataccatcagcattcagcctggtcgtgctgcgtattcgtcgaagacgttgcgcgcattatcaaaacgcatgtattccacggatgacgatttacacgatgcaagaaagcatgtttttggtgtagatgattcatggcgtcctccacagcctgcaattggggcgccattgggtaatccgtcagttgatcgagtcgcgaaaattgtcaatcgttggcttcttgcatgccagtcccggtggggaaacccgttgtctatccaaatcgaacatgtacgagatgcgttgtcttcggcagcgactgcaaccgctgacaagcgtgcatatgaacgggcgttaggcaagcggaacgccgagaaaatgaaagtcaagaatgagcttcggttgcaaggactcaatgaaccgcatgaatctgatgtccggcgtcaagaagctatcactcgtcaacagggcaaatgcttgtactgtggcgatgatatcacattcagtacctgtgagatggatcacatcgttcctcgaaaggggcatggctctacaaatacgcgcgataatctcgctgctgtatgtattcagtgtaatcggcagaagagtaatacgccgtttgctctatggtgccagactccagaggcaaaaagccgcggcgtgagtcttgaagctgcaattcatcgcgtgaaaggtttcttcaccgaatcgaaggagctaacagggcggcaggcgaaggttttcaccagctcgatgataatgcgtttgaagcagacgacagctgacgatcctattgatagtcgctcgatagaatcggtggcatggatggctgatgagttgcatcgtcgcatcgattggcatttcaatggagatgcctctgaaagcgaccatggtcgtagagtgctggttgctgtataccaagggcgtattacttctgaagcgcgcaatgtcatgcgtttccaagcgggtggtgatttccactttgttggcggacatggcaaaacacgcctcgatagaagacaccacgcagtcgatgcgtcggtgattgccatgatgactcctgcggcagcacttacgctggcggaacgtatcaatctccgagatagccaacggtgcattggacgtataagagagggggagattgactggaaacagtggcccaacgagcctacagaaaaatatcagcattggcttgataatgggaaacgcctcttcgcattgatcaatgatgcgctggataatgaccgtattccaataacccattggcagcgctatgcgttgggcaattctattgcacacgaagcaacgattcaccctctgcggaagattccactgggcagtgccattgattatgagacaattagtcgagctgcaactcctgccctgtattgcgccttgacgcgttgcccggactattcggtgaatgatggtttgccggagaacaaacagaggcatattacagtgaatggcaaagtttatgggccggaagatgaggtagcgttctttgcttctgaccatgtggagcttgctgtgcaaggtggttcggcagatattgggaaaactatccatcatgctcgggtttaccgttgttactttgttgatcgtaggggacagaaaaagtggttttacgggatgattcgtgtcttccgagttgatttgatacatgcaaggcatgagaacctattcacttatcctttgccctctcaatcaatatcaatgagatatgcggaaacaagaacggctgaggcggtgttatgcggacatgccgaacatgtcggtaacctggtagctggagatgaaatcgaagttccaatgattggaaagctgacaggcaaaatcgatacgtttgcaaaattctttaatgaatctttgaataatgaatatgttgcagaacggtggagcattgatggtttcgatagtgaatcgaagttgttgcttcgcccgctaatgctggctgaagagggcatagcgaattgggaagataactctcacttatctattcccgatgatgtcaagggactcattgctagaggctggcggccatcggtggacacggtatttgcgaagaaaccgcggattgtccgtcgaaatgtcctaggagaacccagatggaagtcgcgttcaggcatgcccgtttcttggcgagtcacaggctctgaggcatag

SEQ ID NO: 76 - DNA, 3216 bp, Loktanella vestfoldensis
  misc_feature (1)..(3216): Lves Cas9 Open Reading Frame
atgcgtcttggttttgatattggaacgaattcgattggctggtggttgtatgcgaccgacggcaacgagatcaccggggtgatcgacgggggcgtgcggattttctcggacgggcgcgatcctaaatccaaggcctctttggccgttgatcgccgcggcgcccgcgctcaacgccgccgccgtgaccgttacctgcggcgcaaggcggcgttgatgaaacgaatggccgccgccggtttgatgcccgccgatcctgtcgcggcaaaggcgttggaacagcttgatccctatgctttgcgcgcttcgggattggatcaggaattgcccttgacccatctcggccgtgccttgttccacctgaaccagcggcgcggctttaagtccaaccgcaagacggacaagggcgacaacgaaagcggcaagatcaaggatgcgacagcacgtcttgatcaggcgatgatagccaagggtgcgcgtacttacggcgaatttctacatatgcggcgcgcttcagccccggacccaaaatgcgtgccgactgtacgtacccgactgtccatcgcaccgcgtgataacgccgaaaaggcagaggcgggttatgacttctacccggaccggcggcatttgttcgaagaatttaccaaactctgggcggcgcaggccgcaaattccccggatattcttaccgatgagctacgcgatgaaatctcggtgatcatctttcaccagcgcccgctgaaaacacccgaggtcggcctgtgcctgttctcaggatctcatggcgttccgcagaatgataagcgcatcccgagcgcgcatccgcagaaccagcgccgtattctttttgagacagtgaacaacctgaaggtggctgcacggggcgaactggcacgcgggctgacgcgcgatgagcgggacacaattgctcatgcgttagataacaaggcgcataccaagtcgctgtccggcatgtcgatgaagctcaaggcgcttggcaagctgatcaagctgcgtcccgaacaatcattcacactggaaactgccaaccgcgattccatcgtctgcgatccggtgcgggccagcctgtcgcatcccgaccggttcgggtcgcgttggtccacactggacgccgaagcacaatgggatttggtgcagcgcatccgcgccgtgcagagcgatgcagaacataacgcgttggtcgcatggctgatcgcgacgcacggacttgaccgcgtgcacgccgagaacgtggcaaatgccccactgcccgaaggccacggccgtctgggaatgacggcgacaaagcggatattggcggcgctggaagccgaagtgatcccctatagcgcggcggtggcggcttgtgggtggcaccattcggatgggcgtaccggcgaggttctgactgaactgccctattacggccagatcctcgaccgtcacgtgatccccggcacatacgacgagaacgacgacgaagtgacgcgctatggccgcatcaccaacccgacggttcatatcggcctgaaccagctgcggcgtttggtgaacaaaattgtcaccgtttacggcaagcctgatgaaatcgtcgttgagctagcgcgcgatctgaagctgtccgaagatcagaagcgcgacgtgcagcgcgatatcaagaagaacaccgaagctgcgattaccagaggtcaaaagatcgaagaattgggctatgcaaacacaggtgccaatcgggtgatgtatcgcctttgggaggaactcggcccggcaatcggcccgcgctgttgcccatattccggcaagccgatcagtgcctcgatgatctttgacggctcctgtgatgtcgatcatatccttccctattcgcgcacgctggaggacggattttccaaccgtactctgtgcctgaaggagttcaatcgccagaaaaccaacaagactccatgggaggcatggggcaataccccggcctgggatgccatcgaagccaacctcaaaaatctgcccgcgaacaaggcttggcgttttgcccccgatgcgatggagcgtttcgagggcgagaacgatttctctgcccgcgctctgaaagacactcaatacctgtcgcgcatcgcccgcagctatctcgatgcgctttacgatggggcggacggcaagagccatgtctgggttgtgcctggccgcctgaccgaaatgctgcgccgccattgggggctgaacagcctgcttcctgataaggatggcgcggtcaaagccaaaaaccgcagcgaccaccgtcaccacgcgatagatgctgccgttgtcgcggctaccgaccggtccttggtccagcggatcagtaaaatggcgcaaagggacgaagtgaatggggccgaagaggttgcccgctccgtccctcctccttgggacgactttcgaaccgatatcaaatcgcaactagaccgtatcatcgtcagccaccgcgccgatcacggccgaattgactttgccgcacggcaaacgggcaacgacagcaccagcggcgcgttgcacgaggcgacggcactctcaattattgacgaccagaacgtcgcagtccgcattccgctcttgtctttgtccgcagcacagtttgaggaaggcgggcggtcaggctgggttcgtgacccgcagctacgcggcgctttgcatttggcaaccaagggcaaggacaaaaaagacttcgaggcggcgctcctatcattcgctgccaagcccgggccatatcacggaatatcaagggtacgtatcgaaaaacctttgcaagatactgcccgggtctacgtgcccgccgatgcgccgattaaggcttaccaaggcggtagcaatcatcgctacgaagtttggaagcttcccgatggtaaagtcctccatcacgttgtttcaatgtttgttgcccatcagggaaacctgacacgcccccatcctgccgcaaaacgaatttatcaattcatgaagggtgatctggtgagacttgaggacagcaagtttggaccagtgatcgcaacggtggagaagttcaacggaaaggggatgattgagctggttccgcataacgaagctaatgcctcggaccgatatcgcaaaaccaaggaagatctctatatccgcctcggcgcaacaacccttctcagggccaaagcccgccgtgtccatgtcgatgaaatggggcgtctgcgcgatcctggcccaccgcaatag

SEQ ID NO: 77 - DNA, 3318 bp, Sphingomonas sanxanigenens
  misc_feature (1)..(3318): Ssan Cas9 Open Reading Frame
atggatatggcgtggcggctcgggctcgatcttggcaccaattcgcttggctgggcggcgctgtcgctcgatgcggcgggggcgccggatgccattctggcagccggatcgcgcatcttcggtgatggccgcgatccgcagtcgggcacgtcgctggcggtggatcgccgcgcggcgcgggcggcgcggcggcggcgggaccggttcaagcaaaggcagcgcgcgctgctgaagcatctcgaggcggacgggctgttccccgccgatcccgaggtgcagcaggcgctggccgcgctcgatccctatgcgttgcgcgcgcgggcgctggacgaggcgctgagcctgcatgagatcggccgggcgctgttccacctcaaccagcggcggggcttccagtccaaccgcaaggcggatcgcggcaaggatgaggatgcgggcaagatcgcgatcggcgtcgatcggctgaaggatgccatcgcggcggcgggcgcgcggacgttcggcgaattcctccgccagcgccgtgcgggcgccaccggcgagaatcagatacccagcgtgcggacgcggctgcgcgccgagacgggcgagggggcgaagggcagcggctatgatttctatcccagccgcgcgctgctgaaagacgagttcgacgcgatctggcatgcgcaggcggagcatcatcccaaggtgctgaccgacgaggcctatcaccgcctccacgagatcgtcttccgccagcgcccgttgagggcgccgaaggtgggcgcctgcaccctggtgccgggcgaagcgcggctgcccaaggcgcacccgctgttccagcgccgccggctgcttgaggaactgaacgcgctgatgatcgtccgcgccggcgcggtcgcggaacggctgacgccggagcagcgcgacctgctgctgctcaagctgaaggacaagggtaaggtcacgttcaagagcctgcgcgagaaggtgctgaagctggacggcgatgcgcgttttaacaaggaaagcgagcaccgcaccgagttgaagggcgatgaggtcgccgcggaaatgggcggcaagacgcgcttcggctccttgtggccgcacctttccacggagcagcaatggacggtgatcgagcggcagcaggcgctggagagcgatgccgacgaggcggcgttccgcacctggctggtcgagacgcacaagctgacagccgagcaggcgagggcggtggcgggcgcgcggctgcccgctgggcatggccgcttcgggctcaccgccaccgcggccctgctcgccgcgttgcgcgatggccgcacgcccgaggggcgcggcccgaatgcgcccgcgaccgaagcgggccgggtggtggtctatagcgaggcggcggcgatcgccggctatcatcacagcgatcaccgcagtggcgaggtcttcacggacgccaagggccgcccggccttgccctattatggcgtgccgctggatcggcatatcgtgccgggcaccgcagaccccgacgagccggatgaggcggcgcgcatcggccggctgaccaacccgaccgtgcatatcgcgctcaaccaactccgtcgcgtcgtcaaccggctgatccgcgtctatggcccgcccgccgaggtcgcgctggaactggcgcgcgaactcaagctgtccgaggatgagaagaaggagcgcaaccgggagaacagccgcaaccgcctcgatgccgagaagcggtcctccaagctcgccgaactcggccagcgcgacaatggcggcaaccgcgcgctgctcaagctgtgggaggaactgaaccccgagaatatcctcgatcggcgctgcatctattcggggcggcagatctcgatcggcatgatcttctcgggcgcggcggaggtggaccatatcctgcctttcgacgccacgctggatgattccaacgccaacaagatcctctgcctgcgcgaggccaatcgcgacaagcgcaagcgatccccgttcgaggcgtggggcggcaccccgcaatgggaagagatcgccgagcgcgcttcccgcctgccgcgcaacaagcgctggcggttcgagcccgacgcgatggagcgcttcgccgaggagggcggcttcctcgcccgccatctcgtcgacacgcaatatctcggccggatcgctcatgactatctgcgctgcctctatcccgacaagggagacggcagcagccatgtgtgggtttcgccaggccggctgaccgagatggtgcgccgcaagctggggctgaacggtctgctcggcgaccataatctcggcgccgaacagcccaagaaccgcaaggatcatcgccaccacgcgatcgacgcggtcgtcactgcgatcctcgatcgctcgatgctccagcgtatccagcgggcttcgggcgagggggcgagcgatgccgagctgctgcgcatcatcgtgcccgaaccctggacggggtttcgggacgacctgcaacgcgcggttgaccgcatcgtcgtggcgcaccgtgcggaccatggcacggtggccaaggccgcgacgcggggacgggaccagaccgcggcccggctgcacaacgatactgcctacggcttcaccggcgaggcggatgccaagggcacgccgattgtggtccatcgggcgccgctgggggcgctcaaaaagcccgagcatatcgatcaggtgcgcgatccgctgctgcgcgcggcattgcacgatttcacggcggggctgagcggcaagcctttcgaggatcgcatcgccgccttcccccggcttgggccgctcgactatcgcggcatccgccgggtgcgcgtggtggagccgctgcaggtgatcccgatccgcgacgccgccggccgcgcctacaagggctataaaggcgattccaactatcgctacgatgtgtgggaactgcccgacggtaaatgggagcagcgtgtgctgcaaatgtactacgcgcatcagtccggcgagccaccgcgcccgcatccagcggcgcgcaaggttctgagcctgcaccgggacgatgtgctcgcgatcgagcgaggggagggggggcgagaactcgtccgcgtcgtgaaattctcgaccaatgagttcacgctagcgccgctgaatgagggcggggcgctgaagtcgcgtcatgcggacaagggagatccgttcagatatctttatccctcaccctcgactttgaaagcgtggcgcgcacgggaggtgcgcgtggacgaactcggccgggtgctcgatcccggcttccccgcgcgcaagcggcggcgggtcacgcggcccggccgcgcggacgcggattga

SEQ ID NO: 78 - DNA, 4200 bp, Epilithonimonas tenax
  misc_feature (1)..(4200): Eten Cas9 Open Reading Frame
atgacaaaaaatattcttggattagacttgggagtttcatcaatcggttgggcttatgttcaggaagatgataaaaattctgcgaataataaaatcatcaagttaggagttcgtgtaaatcctttgactgttgatgaacaaataaatttcgaaaaaggaaaaccgattacaaccaatgcgggaagaactttagcaagaggagcaagaagaaatctgcaaaggtttaagttgaggagagctaatgttattgatgttttgacaaagggaaatatcttgaaagatggtgatttgcttacagaagttgggaaaaactctacgtttcaaactcaggaattaagagcaaaatctgcgaaagaaaaaatcgaactttcagattttgtgagggttttacttttaattaataaaaaaagaggctataaaagcagtagaaaagcaaagaacgaagatgaaggacaaatcattgacggaatggcggttgctaaaaaattatatgaagaaagcctgactccaggagaatattcttaccaacttttaatagaagggaagaagcaattgccagatttttatcgttctgatttacaatctgaatttgataaagtatggaaatttcaaaagcaattttattctgaaatcttaattgatgaactttataaagaactacaagcaaaaaataaaaatgcgacgtgggcaattttgaaagaaccgttttctcttgttggaatcaaacaaatgggaactatgcaggagaaaaagattgaaaaatatctttggagaagtgaagctgcaaaaaaacaattggattttgaaagcttagctgtcgtgtttcaagagattaacagtaacctaaataattctagcggctatctcggcgcaataagtgatcgaagtaaagaattgtattttaatcatatgactgttggtgaatatctttatcaacaacttaaagcaaaccctcataccaaacttaaaaatcaagttttttatcgacaggattatttggatgaatttgaaaaaatatgggagacacaatctcaatatcattcagaattaaccaaggaattaaaagaacaagttcgtgatgtcgtgattttctatcagagaaaactcaaatcccaaaaaggtttaattagtatttgcgaatttgagaacagagaaattgaaatcatagaaaacggaaaaacaaagaagaaaacagtaggattaaaggttgctcctaaatcttcgccattgttccaagagtttaaaatttggcaagttttaaataatctgcaatttcaaaatttagaaacaaaagaaattttcccaatcgatttagatttcaaacaatcaatttttgatgaagttaatgtcaaaggaagactttctgcaaaagaggttttagatattgtaggttattccggtaaagaatggaaaactaattttaaagatattgaaggcaataataccaatgaaaatctatacactgcttttctgaaaattattgctaatgaaggaaaagaattcccaaaagagtttaagttaacgattgaagacgatattaaagttactaagattcattcttctgcaagtaaaataaaagaatttgtaaaagagaatttttcgtcattaggaataaatacatcaatattagattttaatccagaatttgacggaaaagattttgagaagcaaagttcctatcagctttggcatttattgtattcttacgaaggcgatgattctgcttctggtaatgaaaaattatatgagcttctggagaagaaatttagctttaaaaaagaacattccaaaatattggcagaaattggtttctctccagattatggaagtttgagttcaaaagcgatgcgaaagatttgcacttatatcaaagagcataaatacagcgacgcttgtaatttagctggttataatcactctaaaaattcattgactaaagaacaattagcaaatagaattttaaaagaaaaactagaaattcttccaaaaaattctttgagaaatcctgtggttgaaaagattttgaatcaaatgataaatgtggtcaatgaagtatccaaagaatacggaagaccagacgaaataagaattgagctagcaagagaactgaaaaaaaatgcagaggagcgtgcaaatatgacttctgaaattggcaaagcaaccttgcttcatcaaaaatatgcagaaatattacagaaagaatatgggataaaagtaccatcaagaaacgatattattcggtacaaactgtatttggagctggcaaataacggttttaaagatttatacacaggtcaaaaaatagaaaaggaaaacatttttaccgacaaatatgatattgaccatattatcccgcaatctcgattttttgatgacagtttttcaaataaagttttggtaccgagaggtgcaaatcttaaaaaaggaaacgcaactgcatttgattatttggaaatggaagggaaagatcaactggaaaaattcctcaacaccatcaaagatttgtttgataaaagtttgatttctaaagctaaatttgaaaaacttcagaaaaaaggaagtgaaattggagatggttttatacaaagagatttacgagatacacagtatatagcgaaaaaagcaaaagagattcttttcgaaattaccaattctgtggtttctacatcaggaagaatcacagataaattacgtgaggattggaatctcgtcaacacaatgaaagaacttaatctcgataaatacaggaaattaggtttaacggaaacggtaattaattctaaaggagaagaaaaagaaagaattacggattggagtaaaagaaatgatcatcgccatcacgcaatggacgctttgacagtagcttttacgacgcataatcatatacaatatttgaatcatttgaatgctagaaaagatgaaaagcataatcagcatatcattatttcaaacattgaaaatcttattacaaaagtctatgaaaagaaaaatggttctactaaaagaaagtttgtagaaccgattcataattttagaattgaagccaaaaagcatttagatgaaatattgatttctcacaaaacgaaaaataaggttgttaccaaaaacatcaataaaaccaagaaaaagggtggagtagttgctaaagtagtgttgacaccgagaggtcaacttcataaagaaactatttatggaagctcgaaatttcttaaaactaaagaagaaaaagtatcggggaaatttgatttggaaaccattaacaaagttcagaatgagaaatttagaattgctttattagaaagattaaaagaatttaatggagattctaaaaaagcatttacaggaaaaaatgtgttggcaaaaaatccgatttatttgaatgaagaaaagactgaacaagtttctgaaagtgtaattctggcttggtacgaaaaggcttataccattaggaaagcagtaaattctgataattttaaagattataaaaaccttgaaaaagtaattgataatggcgtaaaagaaatcttaaaaaatcgtctggatgcatttaagggtaatgcaaaagaagcattttctgatttagaaaaaaatccgatttggttgaatgagtccaaaggaatagccataaaaacagttaccataacgggaatcaataatgcagaaactttgcattacaaaaaagaccattttggaaaagaaattctagatgaaaatggtaaaagaatagccgttgattttgtaagtactggaaataatcatcacgttgctatttatgaagatgcagatggaaatttgcaggaaagagtagtgagtttctacgaagctgttgaaagagtgaatcaggggctttcaattatcgataaagaatataattctggattaggatggaagtttctttttacaatgaagcagaatgaaatgtttttgtttccatcagaagattttaatccaaaagaaaatgatttatttgatgaaaagaatctgagtttgatttctaagaatatgtttagagtacaaaagtttggggaattatctaagtcaggtttttggtttagacatcatttggaaacatcagtggaacttaaaaaagaattgagaagtacttcttatttagatttttacagtaaagattttatgaaaactattgttaaagtaagattgaatcatcttggaaaaatagttcaaataggcgaatattaa

SEQ ID NO: 79 - DNA, 4362 bp, Sporocytophaga myxococcoides
  misc_feature (1)..(4362): Smyx Cas9 Open Reading Frame
atgaaaacagttcttggtcttgatttaggtacaaactctattggttgggcattgattcaacatgattttgatagtaaaaaaggtgaaatacttggaatgggtagccggataattccaatgagtcaggatattttaggtgaatttggaaagggaaattctgtttctcaaacagctgacaggactaaattcaggagtgcaagaaggctccgggaacgtcatcttttaagacgagagcgtttacatcgcgttttaaatatccttggttttcttcctcgtcattatgccgctgatattgattttgaaaaacgattagggcaattttttgaaggaaaagaacctaaactagcttatgacaacaatcagttcatttttacaaaatcctttggaaaaatgctggctgattttcgtcagcatcagcctgattttttaaaggatgaaaaaagtaatgatttattaataccttatgattggtctatttattatttgcgtaaagaagctttaacaaaaaaaatagagaaggaagagcttgcatggataattctcaattttaatcagaagcgtggatactaccaattacggggagaggaggaagaggagaatttaaacaagttggtagagtttcattctttaaagattatagatgtagttgcggatgaaaaacttaataataaaggtgagacatggtattcgcttcttcttgaaaatggatggacatacagacgttcaagtaaggttccattatttgattggaaagagaaagtcagagattttattgttactactgatataaatgatgacgggtctgtaaaaacagataaagagggaaatgaaaaaagaagcttcagagcgcccagtgatgatgattggactttactgaaaaagaaaacggaacaggatatcgacaagtcaaggaaaccaattggggcttatatttatgatgcaatacttaaaaaccccaagcaaaaaataaatggtaagcttgtacgtacagttgaacgtaaattctataaggaagagcttaaactgattctacagaagcaaaaggaatttcatcctgaattgcagagtacagatttgtataatgaatgtattcgggagttgtataaaaataatgatgcacatcaattacagttaaataaaaaagattttgttcatctatttttggaagatattattttttatcagcgtccgcttcgaagtcagaaatcttctgttggtaattgtcctttagaattcagaaaatttaaagatagtgaggggattgagaaggtagaatatttgaagacaattcctaagtccaatccatattttcaggagttccgcatttggcagtggatgtataatctttcaatatacaagaaggatgatgatgaaaatgttacccgtgattttctgaaaactatagaagattgggaggatctattcgaatttcttaatcatcgaaaagatattgagcaagagacattgttgaagtttttgttaggaaagaatggggtaaaaggaaaggctcttaaagtagaagcagggaaatttcgttggaattatgtatcagataagatttatccatgtaatgagaccaaagctcttattatttctaagcttgaaaaagtaaaaggtgtagaggagaaatttttgacagaagagatagagtataagctttggcatcttatttattctgtaacagataaagttgagtatgaaaaggctctaaaggcttttgctggtaaacaaaagttggatttggtttcctttgtagattcatttaaaaggtttccaccatttaaaaatgagtatggtgcttattctgagaaagcaattaaaaagattctgcccttattacggacgggaaaatcttggaattggatggctattgatagcaaagtaagggatagaatcaataaaataattactggagaatttgatgaagaaataaagaataaagttcgtgagaaggcggaaaagcatagtttaaagaaggaaaacgattttcaaggcttaccattatggttggcgcaatatgtagtatatggaagacattcagaagcaagtttttcaggtaaatggaactccgttgatgatttaaaaaagtatctcgaagaatttaagcaacattcattgagaaacccgatagtagaacaagtattgacggagactttacgggttgttgctgatatttggcaattttatggaaagggagaaaaagatttctttagtgagattcatattgaactcggaagagaaatgaaaaatacagctgaagaccgtaaagaaatgagtgccataatacaggcgaacgaaacaactaaccttagaataaaagctctattaaatgaactgttgcaagacaagaaggtggaaaatgtaagaccttattctccttctcaacaggaaattttaaagatatatgaagatggcgttttaagttctgatattgaaattccagatgatattcagaaaatcagtaaagcagcccaaccaacgaaatcagaacttcagagatataagttatggcttgagcaaaaatatcgatctccatacactggagcaatgattccattgggcaagttgtttacatctgaatatgaaattgaacatatcattcctcagagtctttattttgacgatagttttagtaataaagtaatttgtgagtcggccgtcaataaacttaaagatagtaggttgggaatggaatttataaaagaatgccatgggatggttgtggaaacaggctttggtaagtcggttactgtttttgaggaagaaacttatagagattttgtggttcaaaattatagtaagaatcattccaaaaaaagtaagcttcttttggaagaaattcctgagaagatgatcgaaaggcagatgaatgacactcgttatataagtaagtttatatcatctgtattatctaatatagtgcgtgaggaggtcaatgatgatggagttaactcaaaaaatattgttccgggtaatggtaaaattacaacacagttaaaacaggactggggtttaaatgatatttggaatgaattgattttaccacgctttgaacgtttgaatgttttgactgattcaaaacattttacagcttggagtgaaaatcatcagaggctattgccaactgtaccgatagggctttctaaaggattttccaagaaaagaattgatcatagacatcatgctttggatgccttggttatagcctgtgcctccagaaatcatatcaattttttgaacaatgcacatgcaatagataaaaagaaaaattcggaggaaaaacaaaaatttagacatgatttaaaagcgattctttgtgataaaaagtatagtgataaatccgaaaagaattacaggtggatattcaagaaaccttgggataattttactattgattcaaaaaacgctttggataaaattattgtaagctttaaacaaaatcttcgaattatcaataaggcaacaaaccgttatgaaaaatgggtagatagagatgggataaaagtaaaagaatggcataagcaagaaggaataaactgggctactagaaagcctttgcataaggatacagtttcaggtaaagttgatttaaaaagggtaacagttccagaaggaaagatattgaccgctaccaggaaaagcttagatacatcgtttgacttgaaggtcattgaatctattacagataccggtattcaaaaaattctaaaaaattatcttactagtaaatcaaataatccggagctcgcattttcttcggagggtgttgaggatatgaataagaatatcagaaaatataatgatggaaaattgcatcaacctatatataaagttagaatatttgagttggggagtaaatttccattgggacaatttggtaataaaaagtttaagtatgtagaaacagcaaaagggactaatcttttctttgctgtatatgaagatgaaaataaaaataggaattatgaaacgattcctttaaatgtagttattgaaaggcaaaaacaaggactctcttctgtgccaataaaaagtgaaaaagggcataaattgttattctatttgtccccaaatgatatagtctatgttcctggtagtaatgaagaattcagtatagataggctttatagatttacagattccagcgataagactgctaattttataccacttagtgtttcaagtttaatttttagctcaaataaaaatgagcaaaaaaaaatagggattagctatccaattcaagatgagtttggtctaggaagtccacagtcaaaaaatcaaaagtcgatcgacggaataatgattaaagagaaatgtgtaaaagtgaatatagacaggcttggtagggtgtcattttga

SEQ ID NO: 80 - DNA, 4530 bp, Psychroflexus torquis
  misc_feature (1)..(4530): Ptor Cas9 Open Reading Frame
atgaaaagaattttagggttagatttaggaacaaactcgattgggtggagtctaattgaacatgattttaaaaataagcaaggacaaattgaaggattaggtgttcgtataattcctatgagtcaagagatactaggtaaatttgatgctgggcaatcaatctctcaaaccgcagatagaacaaaatatagaggcgttagacgattgtatcaaagagacaatcttcgaagagaacgtctacatagagtgttaaaaattttagactttcttccaaagcattatagcgaaagcattgactttcaggataaagtaggtcaattcaaacctaaacaagaggttaaactcaattatcgcaaaaatgagaaaaataagcacgaatttgtttttatgaattcatttattgaaatggtaagtgaattcaaaaatgcccaaccagagcttttttacaataaaggtaatggagaagaaacaaaaataccatatgactggacattatactatctccgtaaaaaagccttaactcaacaaattactaaagaagaactagcctggttaattttaaatttcaatcaaaaacgaggctattatcaattacgtggagaagacatagatgaggacaagaacaagaaatacatgcaacttaaagtcaacaatttgattgattctggtgcaaaagtgaaaggaaaagtattgtataatgtaatttttgataatgggtggaaatatgaaaaacaaattgtcaataaagatgaatgggaaggaaggacaaaggaatttattattaccactaaaacactgaaaaatggtaatattaaaagaacatataaagctgtagactcggaaatagattgggctgcgatcaaagctaaaactgaacaagacattaataaagcaaataaaacagtaggcgaatatatttacgaatctctattagacaatccttctcaaaaaataagagggaaattggttaaaactatagaacgaaaattttataaagaggaatttgaaaagctactttctaaacaaattgaattacaacctgaactatttaatgagtcactgtacaaagcttgtattaaagaattataccctagaaatgaaaatcatcaaagtaataataaaaaacaagggtttgagtatttatttacggaggatattatcttttatcaaagaccacttaaaagtcaaaaatctaatatttctggttgtcaatttgagcataaaatttataagcaaaaaaataaaaaaacaggtaagcttgaattaataaaagaacctataaaaaccatttccagatcacatcccttatttcaggaatttagaatttggcaatggttacaaaatcttaaaatctataataaagaaaaaatagaaaacggaaagttagaagatgtaacaactcaactattacctaataatgaggcctatgttaccttatttgattttttgaacactaaaaaagaacttgagcaaaagcaatttatcgagtattttgtaaaaaagaaattaatagataaaaaagaaaaagagcattttcgttggaactttgtagaagataaaaaatatcctttttctgaaaccagagcccaatttttatcacgcttagccaaagttaaaggaataaaaaatactgaagattttttaaataaaaatacgcaagtaggaagcaaagaaaatagtccatttattaaacgaatagagcaattatggcacatcatatattcggtttctgatctaaaagagtatgaaaaagcactcgaaaaatttgcagaaaaacacaacttagaaaaggactcctttttaaaaaacttcaaaaaatttcctccatttgttagcgattatgccagctactctaagaaagctatatcaaaactattaccaattatgcgcatgggtaaatattggagtgaaagcgccgttccaacccaagtgaaagagcgttccttatcaattatggaaagagtaaaagtcttacccttaaaagaaggttactctgacaaagatttagctgatttgctttcaagagtaagtgacgatgatataccgaagcaattaataaaaagttttatttcttttaaagacaaaaacccattaaaaggcttaaatacataccaagccaattatttagtatatggtagacactcagaaactggagatatacaacattggaaaacacctgaggatattgacaggtatttaaataatttcaaacagcattccctacgcaatcctattgtagagcaagtggttatggaaaccttgcgtgtagtgagggacatttgggagcattatggtaataatgaaaaagacttctttaaggaaatccatgtggaattaggcagagagatgaaaagccctgctggtaaacgagaaaaattatcacaaagaaataccgaaaatgaaaacactaatcatcgtatccgggaagttttaaaagaattgatgaatgatgcctctgttgaaggtggtgtacgcgattattctccgagccagcaggagattcttaaactttatgaggagggcatttaccaaaatcccaacaccaattatttaaaagttgatgaagatgaaatactaaaaatacgcaaaaagaataatcctactcaaaaagagatacaacgctacaaactatggttagaacaaggatatatctcaccttatacaggaaagattattcccttaacaaaactgtttactcacgaatatcaaattgaacatatcataccacaatctaggtattatgataattctctaggaaataaaatcatctgcgaaagcgaagtcaatgaagataaggataataaaacagcttatgaatatttaaaggttgaaaaaggaagtattgtttttgggcataagcttctcaatttggacgaatatgaagctcacgtgaacaaatatttcaaaaaaaataaaacaaaactaaaaaatttattaagcgaagatatccctgaaggttttattaaccgacaacttaatgatagtagatacatcagtaagctggtaaaaggactattgagtaatattgtacgagaaaatggggaacaagaagcaacatcaaaaaaccttattccagtaactggtgtagtcacctcaaaactaaaacaagattgggggcttaatgataaatggaatgaaatcattgctcctcgttttaagcgattaaataaactcacaaattcaaatgattttggtttttgggataatgacattaacgcctttagaattcaggttccagatagtcttatcaaaggttttagcaaaaaaagaatagaccatcgccaccatgccttagatgccttggtggtagcttgtacttcaagaaatcatacacattacttgagtgcattaaatgccgaaaataaaaattacagcttgcgtgacaaacttgtaatcaaaaatgagaacggtgactatactaagacctttcaaataccgtggcaaggttttacaatagaagctaaaaacaacttagaaaaaacggttgtaagctttaaaaagaacctgcgtgttattaacaaaaccaataataaattttggtcttacaaagatgaaaacggaaatctaaaccttggaaaagatggaaaacctaagaagaaacttcgcaaacagaccaaaggttataactgggcgattcgcaaacctttgcataaagaaactgtatcgggaatttataatattaatgcgccaaaaaataaaattgcaacttcagtaaggactttattaacagaaatcaaaaatgaaaaacatttagcaaaaataaccgatttacgtattagagaaacgattctacctaatcatctaaagcattacctaaacaataaaggggaagcaaattttagtgaagcatttagccaagggggtattgaagatttaaacaaaaaaattacgactttaaacgaaggaaaaaaacatcaacctatttatagagtgaaaatatttgaagtaggcagtaagttttcaatttcagaggatgaaaactctgcaaaaagtaagaaatatgtagaagctgcaaaaggcaccaacttgttctttgctatttatttggatgaggagaataaaaaacggaactatgagaccattccgcttaatgaagtaatcacccatcaaaaacaagtagcaggttttcctaaatctgaaagattatctgtacaacctgattctcaaaaaggcacattcttattcaccctttctcctaatgatttagtttatgtaccaaataatgaggaacttgaaaatcgtgatttatttaatttggggaatttgaatgtcgaacaaataagtagaatttacaaattcactgactcaagtgataaaacttgtaattttataccatttcaagtatcaaaattgatatttaatttaaaaaaaaaggagcaaaaaaaattagatgttgattttattattcaaaatgagtttggcttaggaagtcctcaatctaaaaatcaaaaatcaattgatgatgttatgataaaagaaaaatgcattaaactcaaaatagacagattagggaacatttcaaaagcctag

SEQ ID NO: 81 - protein, 1368 aa, Lactobacillus reuteri
MIKKDYNIGLDIGATSVGFAGIDEQYDPIKLKGKTVVGVNLFEEGQTAADRRSFRTTRRRLNRRKWRLSLLEEFFDPYITPVDPAFFARLKESNLSPKDNNKNFSRSLLFPDITDQKFYEEYPTIYHLRYALMTENKKFDLRAIFLAIHHMIKYRGNFLNSTPVAHFDTSKIDFANDFSKLNRLYLNEDPNNIFEINLQNVKEISDILLDHSIKKFDKQKQVAKLLLTSQNDKELDKRNKQIATQISKAILGYNFSLNEILKLEAVNKSKWKLNFSSADIDDTLPDLISELDESQESILNIILSLYSRLTLNGIVPSGMSLSESMIDKYGTHKEHLDLLKKYLKTLPIKNRKEIAEAYAEYVGNSLKKSGHISQEEFYKAVKKNLDKSETAQKILSLISEEKFMPKQRTNQNGVIPYQLHQKELDQIIVNQSQYYPWLAELNPVTEHKDAKYKLDELIAFRVPYYVGPLIDPKTIPQTEQGNKNASFAWMVRKENGQITPWNFDKKVDRISSANNFIKRMTTKDTYLIGEDVLPAHSLIYERFKVLNELNMIRVNGKKLSVSVKQNLYNDLFKQQKTINRKKLANYLQANLGIPERPQITGLSDPEKFNSQLSSYIDLQKILGSEIVDDPNKQDDLEKIIEWSTVFEDSRIYKVKLQEIGWFTEKQKNELVSHRYQGWGRLSKKLLVELKDKNGRSIIDLLWNSQRTFMEIQSRPEFAEQITNENQDKLTEDNYEDVLADAYTSPQNKKAIRQVIKVVDDIVKATGKAPKFISLEFARSDERSDRVKSRKTHIQKIYETTAKELLKDDQLIKELGSVSDLSDRLYLYFTQLGRDMYTGKPINIDEISTMYDIDHILPQAFLKDDSLDNRVLVRRQDNNAKSDTVPALKFGKMKPFWNKLQKHGLISKRKLNNLQTNPESIDKFKAVGFVNRQLVETRQVIKLAANILASRYPDSKIIEVKASLTHQMRESFNLIKNRDVNDYHHAVDAYLSAFVGQYLYNRYPKLQPYFVYGQFKKFDKQSTRIGMKTNHFNFLYDLEPEGKNVKIKKPTKIINKETGEIIGDRDELVAKLNRVYNFKYMLVSQEVYTRSGALFDQTIYPANSGKKLIPLKQNKTTAIYGGYSGSKAAYMSIIRLRDKKGGTYRIVGIPVRAVNKLNQAKKKSNEKYLAELKAVIEPQIAKTKKDRKTGQRVLVPQEFDVIIPEVMYRQLIVDGDQKFTLGGTIDRYNAVQLVLNQEILTFLEQPTKYKDADTKLLDIYDQIVNLVEKYFMLFDSKRLAAGRVAFEKLPTLQPVDKMPSKLIIIRRIIQGLHDNAARTDLKAINGSSSFGRLQKRNGIILSPNACLIYQSPTGLFERKVYLNTISPLK

SEQ ID NO: 82 - protein, 1369 aa, Lactobacillus rossiae
MDKSKPYGIGLDIGTNSVGFVATDAEGHLIRLKGKTVIGAYLFNAGISAAERRGFRTTRRRLSRVKWRLGLLREIFETHFQESMGENEDNDFFLRFKYSNISPKDPQFSTAKGLFNDRTDKEFYDQYPTIYHLRRALMTEDHQFDIREIYIAMHHIVKYRGHFLKEGRAKDFKVGDLRLLDNFKMMNEQIEEINPLWQLKLPTDDASIKSITAILLDNTQSQNDRQKAVTKVILATLVKASDKDINAARKRFVGELSKAMVGLKTKLWVLADVSQNGDWEIKYENYADFAETIGSGESDTIQSLFNEINDLYGVITLAGIIPKEAESFSDGMVRKYEHHRKNLELLKVYCAEQSDGKRGRQIRQTYDKYIDGVDSKQFTQEDFYKALSKFTAKDEATSENAKLIAQEIAVGTFMPKLRTKANGTIPHQLHQKELDAIIENQKKYYPWLGEVNPVESHRRALPYKLDELVSFRIPYYVGPMVTPTKGDPEKSKFAWMVRKEPGTITPWNFDQKVDRSASGEAFIQRMKTTDTFLIGEDVLPQQSLLYQKFEVLNELNKIMINGKPICREQKQRLFKQLFMQYKTVTVKKVQQNLIANGEESENVPITGLSDPLRFNSSFSTYIDYKDILGTAAVNDNAKQSDIEQIIAWSTIFEDAAIFREKLNDITWLNDDQRNKLSHKRYRGWGRHSRKLLAGLRDGEGQTIIERLWNTNDNFMQIQNDSEIARQITEANSSKMATAEGTDEIIDGFYTSPENKKALREVMKVVKDIQRAHHGQAPAWVYIESPRETPRPGQRTVSREQQLTDLYEGAAKEIVDDAVLNELKDKVKSKENFTDKLVLYFLQNGHDIYANDSINIDNLNAYDIDHVLPQSLIKDDSLDNRVLTTHERNLKKSNRFATELFADQRKKWEKWHRLGLISSRKLKHLTMQPNSVEKFAHGFIARQLTETRQIIHLTANVLSNLYQENDTKIVMIKAGLNSEFRRTFDFPKNRSVNDYHHAFDAFLTAKIGRYLLARYPKLEPFFVYGNFVKNPKAMKRLSSFDFIAQLAAKTDDTSHIDQRSLKQVPVVNEETGEIVWDKDIELAELDKTYNYKTMLVKRAQTENNAQMFKQTVFKARDNQNKTLIPVKNGLSTDVYGGHSQQAISYLCIVWVGQKKKYRVLGISTAHAGILNNFEKNYGRFEAKKKLQEIVSNTLDNADRNDFKIVAPKVLFEQVVEDDNMKFGLGSASDYRNVQQLFLSRKNQLLLANMMTDQIHDQDLVHLFDEIVGQMNAHFPIFDRGGYRSSLTQSRDKFLKLPFKKNEDLITKQEVIRRILDGLHANANRKDLKIIGSKGDFGRLGTKKIYLSKDAKLIYTSPTCLFTRTVPLSSL

SEQ ID NO: 83 - protein, 1346 aa, Pediococcus pentosaceus
MEKVPYNIGLDIGTSSIGFAATDNLNKPIRAKGKTVIGVRLFEEGKTAADRRGFRTTRRRLSRRKWRLRLLDEIFDKEMAKVDNTFFARLKESNLSPKDANKKYLGSLLFPEKKDFKFYEDYPTIYHLRYALMHEKRQFDIREVYLAMHHIIKYRGNFLNSAPMNSFKTQDFDFVAKFEKLNELFESIDAEHETKFDIENISKFRDIMLNQDIRKLDRKKQAAKILILDSTDKTAKKINNKIATAVANSALGYKFALDAILKLDVEESKDWSISLNDEEIDSILDNLTSDLDAERIEIIEILRDLYSHIALNEIVPNGQSLSKSMMDKYDKHHADLDVLKKVISNMDDRKKAKSLKNIYNQYVGKTNDKVLDKDEFYKQIQKNLDESEDAMKIVNEIELDQFMPKQRTSQNGVIPHQLHQKELDEIIENQKQYYPFLAEPNPNEKRKPHAQFKLDELIAFKIPYYVGPLITKEEQQAQSGAKFAWMKRKQDGVITPWNFDEKVDRMASANEFIRRMTTKDTYLLGEDVLPDESLIYQKFKVLNELNNVKVNDKKLTVSDKQDIFNDLFKKQKTVSVSKLQKYFVTEKHYLTEPTIKGLSDTKKFSNSLSTYIDFEKIFGNEILADQNKQNDLEKIIEWSTIFEDRKIFEDKLHEIEWLTEKQIKAVRRYRGWGRLSKKLLVDLRNNEGKSILDELWRTNDNFMQIQAREEFAKSIVEANQKLMNLGGAASVQNTVESTLEDAYTSPQNKKAIRQVIKVVEDIVKAVGYAPEKITIEFTRGADKNPRRTQNRQKQIMEVYKTAAKEIVDATLKGQLENEEKLTDKLYLYFTQLGKDIYSGETINIDQLNNYDIDHILPQAFIKDDSLDNRVLTSRDLNNGKSDSVPVKQFGANMKSFWMRLQAHGLISKRKLNNLMTDPDSIGKYTMQGFVRRQLVETSQVIKLTANILGAIYGENTDIVEIPAKLTHQMREKFNLYKVREVNDYHHAFDAYLTTFVGNYLFKRYPKLRPYFVYGDFKMTDNALKGMRRFNFLHDLKDDEVLVDNETGEVLWEGQKSIEELKKIYGYKFMLTTHEAYTQHGPMFKQTVYSSDTPGKLIKIKNNKPTEIYGGYTSNTDAYMAIVRIKARKGDTYKVVGVPRKEGDALSRIKLLDESKYHENLKNILAINLNKSLNKFDVVLDKVKYRQVIYDGTDHLMLGSSKYKYSTKQLVLSDQSMKILSSTGEFSDEELIKVFDEIMYIVNKNFSLYDTRGFRDKLNNARENFIKLPNKTLFEKGKLKQHSKLEILKQILIGLHANAGRGDLKDIGVNNFGAMVVTAGVTLSPDATIVYQSPTGLFERKVKLSDL

SEQ ID NO: 84 - protein, 1130 aa, Lactobacillus nodensis
MENKISLGLDIGVASVGFSVIDAQEGKVLELGARLFNSSVSAENQTRRDMRGSRRLSNRKKQRRKDVAQLFKTFGLINYFDKENYFDNFQNNLNSYELRVKGLSEKLSKEELVNSLYHIVKRRGISYDLADADTDFDGSDYSSSLNQNQLELQTKTPAEIQLTRLNVHGAVRGKVTINGEDEDTMQVLLNVFPTKSFVSEAKKIIQTQQQYYPDILTDIFETKYLEILERKREYFVGPGSEKSRTDFGIYKKDGRTLDNLFEELIGHDKIYPDELRASGASYTAQVFNVLNDLNNLRISSYENGKISTEDKIKIVEDLRNNIGNVIIMKIIKKVAGCEDDDIKGYRLDSKDKPDIHSMAVYRKVHRDLLKYDVDIIKWPTEFIDELSPILTLNTENGEIRKQMVNKLQPKYSFLTDELIQVIINNKSSFDVTSNNKWHRFSLKTMNVLIEEMFRRPVEQMTLIQELGLIKDSGKRFENCKLLPYREISKDIFNPVASKSVREALKIVNAVMKKYGQIDYLVIEMPRDKNEEEMKKQIEKFQKENNKQKDEAINEFVKKIGNKNAVDDGLRRYGGKLYFKIRLWYQQDGIDLYNGKVIEPFDLLNNINKFEVDHIIPESISFDDSINNKTLCYADMNQIKGQKTPFEFMNEGHGQGFAKMKAMVNKNSKLKGKRKNYLFDENISDIETRKRFISRNLVDTQYSSRVVLNSLQEFFKEKETGTKVTVVRGKFTSNLRKHWHINKTRDTFHHHAIDASIIAATPFLRIWKKDASLFPMHVSENTVDIETGEILNDTEFKKDFYGLPYSSFIEELNGADDRIKFSHQVDRKMNRKVSDATIYSTRKGMLNKDKEETDYVLGKIKNIYDVSEYNKFKRIYDKDPNKFLLAHHDPKSFDELRKIMQEYPSKIDKVMTNGKVKSVDISPFELYRRKHGMVQKYSNKNKGPVIKQLKYLDKKLGSHIDITPKDTLNDRHVVLQSLKPWRTDVYYNSVTGEYEIMGIKYSDLKFNGGEYGIKMSKYLEIKEREQVSDESEFLFTLYKRDRIQIINCENDEIVEMLFWSRNNSNIGYAELKPVYKYKTEDESWPVYGYGKNQILKRLVPKNCKILKVNTDILGNPYYIKKESKNPKNILD

SEQ ID NO: 85 - protein, 1361 aa, Sulfurospirillum sp.
MTSLISLDLGGKNTGFFSFTAKDVSIIDTFQSGTIIYDESFVLSQVARRGKRHGKRNNLRNTLVKRLFLLLLQKHYGLSLDFLPDEILGLFNKRGYTYASFEIKEDEKENLESDILKEFLNDKLNYTIQNDDEVEEFLNQIASNEETFKNYKKDFENLFGASTHQPKKQIELIDEIKKDLEKEDAKELLDGLKVIKKIIDEFHKQQNQGNLPRAKYFEELYLEIEYNLKIQKFFTCNHLHINDMQYLIGNLSNYQLKELRRYFNDEAMAKEDFWSCEKLHRITWRFIQSWHPKSPEDKQRQKENLANLKTKSIIEFLTTTNPLMTIPPYDDMNNRGAVKCQTLRLNEEYLDKHLPHWRAIAHTLASETQKENLEGVTVKGYSEDSTLLHRILDTSSIIDPYRLRSDEIDSYCDVLTKDNAFALKKFAKEYYQLVKEKVRTGIWTKDDDMFKKCDHNPPHKNNQIHNLVAGILGKPIAKERFEAFENELWNVKFGNKKLSSYCKNIEEFRKSNGNLFKQIVELGEDKEVQKYQKELNEWVRKIGEFFNIETPYRARFNNLFSMAQLHTIIDTTRSGFNATCKWCSCENQYRASTRIEIDEQTGEITTNANCQRLPADTQRPFSGKIERYIDKLGYEIAKVKAKELEGIKEDTIDLKIILEQNAFAYEESIRNAKIKNANAKAKKALEEAQKRGLKNIEDKTKRIKDFSNSICPYCGQSLGEDGEIDHILSRSYTLKKYDTVFNSEGNLLYVHQKCNQAKLAKTDYSLQDLKIDISQKWIEEQIATIKTYKTFSVLTQEQQKAFKYALFLDNSNEAYQKVISWLRTDQSSRVNGTQKYLAKKIQEKLKAMFPAKTFNFEFILADANDVHDLRIKAYQLPEKPKDSKQETYSHTIDAVMSLVSVWDKVLPKTEKPTKEDILKFANVENWSALNNEFLTKGKSANQKIEEMIQANDFGQKNMRQVFSKPIFKDESIGERYKPFVRYHNQFYIGYPISIKDGYDMQHCQAMISKNDISRVEEILKDTSLCTLLKEKNGIKLYSINKQSINELSNQFFNLNYQNLNDAQKKKSELAEFVINHCKYYVKKTSVINAPQFIDKDSMKPYPFYKDWQKFHEAYKKELDAEPKTKKDNGKLVYDISGIDDFWTEFCKKYFGIKTKDNRNKARKVFSIVALTSAPGTVFRIKRKTPKGHIYQATAIDNQQISGDYANVLLAGNSKTLALAGQKPSSDLKKELSVKESKDIRDIKLEPSRFFKEGFDCRGIEVIVNKTSATIKNFPLTKIDKKIKKLIFKTLFEKKDGKRQKQKTSISLKEKNTMQETLKKLLKDSIKVTIRDGSISGIEISKKTVNFTLPFKSENLAKLLDD

SEQ ID NO: 86 - protein, 1147 aa, Bifidobacterium thermophilum
MSDKTYRIGIDVGLYSVGLSAIQVNDDDDPVRILNAQSVIHDGGVDPNAQKSADSRRAQSGIARRTRRMRRNRKKRLKRLDQILVESGFPVSSENDLEGFEPWLLRAQAADAFIEDEDIRKRAISVSCRHIARHRGWRNPYLDVRTLLAVDSPSSAFYDKLVENAALEMDGQMPDSDATPAQIVRDVLEYKRGEAAIRLRKSTAENKKNRLALFPEKMMQDDYAYELRLILAKQAVPKDIARKLILAVFQSQSPKGSAEKRVGKDPLDPSQPRALKASLAFQEYRILNILTNLRLQDGGAERRLSIEEKQKLYKMLVEDTGREKKYETWTDIASAMEWKRNWLKGVGSLTADGDDRVTSRPPHIDIVEKLNGIKDTKFRKSILSWWKSATDVNREAMIALLSNTVDIAKKQDDPDFSSAVDFIDSMDDSDLQILDTISIQPGRAAYSSKTLRALSKRMYSTDDDLHDARKHVFGVDDSWRPPQPAIGAPLGNPSVDRVAKIVNRWLLACQSRWGNPLSIQIEHVRDALSSAATATADKRAYERALGKRNAEKMKVKNELRLQGLNEPHESDVRRQEAITRQQGKCLYCGDDITFSTCEMDHIVPRKGHGSTNTRDNLAAVCIQCNRQKSNTPFALWCQTPEAKSRGVSLEAAIHRVKGFFTESKELTGRQAKVFTSSMIMRLKQTTADDPIDSRSIESVAWMADELHRRIDWHFNGDASESDHGRRVLVAVYQGRITSEARNVMRFQAGGDFHFVGGHGKTRLDRRHHAVDASVIAMMTPAAALTLAERINLRDSQRCIGRIREGEIDWKQWPNEPTEKYQHWLDNGKRLFALINDALDNDRIPITHWQRYALGNSIAHEATIHPLRKIPLGSAIDYETISRAATPALYCALTRCPDYSVNDGLPENKQRHITVNGKVYGPEDEVAFFASDHVELAVQGGSADIGKTIHHARVYRCYFVDRRGQKKWFYGMIRVFRVDLIHARHENLFTYPLPSQSISMRYAETRTAEAVLCGHAEHVGNLVAGDEIEVPMIGKLTGKIDTFAKFFNESLNNEYVAERWSIDGFDSESKLLLRPLMLAEEGIANWEDNSHLSIPDDVKGLIARGWRPSVDTVFAKKPRIVRRNVLGEPRWKSRSGMPVSWRVTGSEA

SEQ ID NO: 87 - protein, 1071 aa, Loktanella vestfoldensis
MRLGFDIGTNSIGWWLYATDGNEITGVIDGGVRIFSDGRDPKSKASLAVDRRGARAQRRRRDRYLRRKAALMKRMAAAGLMPADPVAAKALEQLDPYALRASGLDQELPLTHLGRALFHLNQRRGFKSNRKTDKGDNESGKIKDATARLDQAMIAKGARTYGEFLHMRRASAPDPKCVPTVRTRLSIAPRDNAEKAEAGYDFYPDRRHLFEEFTKLWAAQAANSPDILTDELRDEISVIIFHQRPLKTPEVGLCLFSGSHGVPQNDKRIPSAHPQNQRRILFETVNNLKVAARGELARGLTRDERDTIAHALDNKAHTKSLSGMSMKLKALGKLIKLRPEQSFTLETANRDSIVCDPVRASLSHPDRFGSRWSTLDAEAQWDLVQRIRAVQSDAEHNALVAWLIATHGLDRVHAENVANAPLPEGHGRLGMTATKRILAALEAEVIPYSAAVAACGWHHSDGRTGEVLTELPYYGQILDRHVIPGTYDENDDEVTRYGRITNPTVHIGLNQLRRLVNKIVTVYGKPDEIVVELARDLKLSEDQKRDVQRDIKKNTEAAITRGQKIEELGYANTGANRVMYRLWEELGPAIGPRCCPYSGKPISASMIFDGSCDVDHILPYSRTLEDGFSNRTLCLKEFNRQKTNKTPWEAWGNTPAWDAIEANLKNLPANKAWRFAPDAMERFEGENDFSARALKDTQYLSRIARSYLDALYDGADGKSHVWVVPGRLTEMLRRHWGLNSLLPDKDGAVKAKNRSDHRHHAIDAAVVAATDRSLVQRISKMAQRDEVNGAEEVARSVPPPWDDFRTDIKSQLDRIIVSHRADHGRIDFAARQTGNDSTSGALHEATALSIIDDQNVAVRIPLLSLSAAQFEEGGRSGWVRDPQLRGALHLATKGKDKKDFEAALLSFAAKPGPYHGISRVRIEKPLQDTARVYVPADAPIKAYQGGSNHRYEVWKLPDGKVLHHVVSMFVAHQGNLTRPHPAAKRIYQFMKGDLVRLEDSKFGPVIATVEKFNGKGMIELVPHNEANASDRYRKTKEDLYIRLGATTLLRAKARRVHVDEMGRLRDPGPPQ

SEQ ID NO: 88 - protein, 1105 aa, Sphingomonas sanxanigenens
MDMAWRLGLDLGTNSLGWAALSLDAAGAPDAILAAGSRIFGDGRDPQSGTSLAVDRRAARAARRRRDRFKQRQRALLKHLEADGLFPADPEVQQALAALDPYALRARALDEALSLHEIGRALFHLNQRRGFQSNRKADRGKDEDAGKIAIGVDRLKDAIAAAGARTFGEFLRQRRAGATGENQIPSVRTRLRAETGEGAKGSGYDFYPSRALLKDEFDAIWHAQAEHHPKVLTDEAYHRLHEIVFRQRPLRAPKVGACTLVPGEARLPKAHPLFQRRRLLEELNALMIVRAGAVAERLTPEQRDLLLLKLKDKGKVTFKSLREKVLKLDGDARFNKESEHRTELKGDEVAAEMGGKTRFGSLWPHLSTEQQWTVIERQQALESDADEAAFRTWLVETHKLTAEQARAVAGARLPAGHGRFGLTATAALLAALRDGRTPEGRGPNAPATEAGRVVVYSEAAAIAGYHHSDHRSGEVFTDAKGRPALPYYGVPLDRHIVPGTADPDEPDEAARIGRLTNPTVHIALNQLRRVVNRLIRVYGPPAEVALELARELKLSEDEKKERNRENSRNRLDAEKRSSKLAELGQRDNGGNRALLKLWEELNPENILDRRCIYSGRQISIGMIFSGAAEVDHILPFDATLDDSNANKILCLREANRDKRKRSPFEAWGGTPQWEEIAERASRLPRNKRWRFEPDAMERFAEEGGFLARHLVDTQYLGRIAHDYLRCLYPDKGDGSSHVWVSPGRLTEMVRRKLGLNGLLGDHNLGAEQPKNRKDHRHHAIDAVVTAILDRSMLQRIQRASGEGASDAELLRIIVPEPWTGFRDDLQRAVDRIVVAHRADHGTVAKAATRGRDQTAARLHNDTAYGFTGEADAKGTPIVVHRAPLGALKKPEHIDQVRDPLLRAALHDFTAGLSGKPFEDRIAAFPRLGPLDYRGIRRVRVVEPLQVIPIRDAAGRAYKGYKGDSNYRYDVWELPDGKWEQRVLQMYYAHQSGEPPRPHPAARKVLSLHRDDVLAIERGEGGRELVRVVKFSTNEFTLAPLNEGGALKSRHADKGDPFRYLYPSPSTLKAWRAREVRVDELGRVLDPGFPARKRRRVTRPGRADAD

SEQ ID NO: 89 - protein, 1399 aa, Epilithonimonas tenax
MTKNILGLDLGVSSIGWAYVQEDDKNSANNKIIKLGVRVNPLTVDEQINFEKGKPITTNAGRTLARGARRNLQRFKLRRANVIDVLTKGNILKDGDLLTEVGKNSTFQTQELRAKSAKEKIELSDFVRVLLLINKKRGYKSSRKAKNEDEGQIIDGMAVAKKLYEESLTPGEYSYQLLIEGKKQLPDFYRSDLQSEFDKVWKFQKQFYSEILIDELYKELQAKNKNATWAILKEPFSLVGIKQMGTMQEKKIEKYLWRSEAAKKQLDFESLAVVFQEINSNLNNSSGYLGAISDRSKELYFNHMTVGEYLYQQLKANPHTKLKNQVFYRQDYLDEFEKIWETQSQYHSELTKELKEQVRDVVIFYQRKLKSQKGLISICEFENREIEIIENGKTKKKTVGLKVAPKSSPLFQEFKIWQVLNNLQFQNLETKEIFPIDLDFKQSIFDEVNVKGRLSAKEVLDIVGYSGKEWKTNFKDIEGNNTNENLYTAFLKIIANEGKEFPKEFKLTIEDDIKVTKIHSSASKIKEFVKENFSSLGINTSILDFNPEFDGKDFEKQSSYQLWHLLYSYEGDDSASGNEKLYELLEKKFSFKKEHSKILAEIGFSPDYGSLSSKAMRKICTYIKEHKYSDACNLAGYNHSKNSLTKEQLANRILKEKLEILPKNSLRNPVVEKILNQMINVVNEVSKEYGRPDEIRIELARELKKNAEERANMTSEIGKATLLHQKYAEILQKEYGIKVPSRNDIIRYKLYLELANNGFKDLYTGQKIEKENIFTDKYDIDHIIPQSRFFDDSFSNKVLVPRGANLKKGNATAFDYLEMEGKDQLEKFLNTIKDLFDKSLISKAKFEKLQKKGSEIGDGFIQRDLRDTQYIAKKAKEILFEITNSVVSTSGRITDKLREDWNLVNTMKELNLDKYRKLGLTETVINSKGEEKERITDWSKRNDHRHHAMDALTVAFTTHNHIQYLNHLNARKDEKHNQHIIISNIENLITKVYEKKNGSTKRKFVEPIHNFRIEAKKHLDEILISHKTKNKVVTKNINKTKKKGGVVAKVVLTPRGQLHKETIYGSSKFLKTKEEKVSGKFDLETINKVQNEKFRIALLERLKEFNGDSKKAFTGKNVLAKNPIYLNEEKTEQVSESVILAWYEKAYTIRKAVNSDNFKDYKNLEKVIDNGVKEILKNRLDAFKGNAKEAFSDLEKNPIWLNESKGIAIKTVTITGINNAETLHYKKDHFGKEILDENGKRIAVDFVSTGNNHHVAIYEDADGNLQERVVSFYEAVERVNQGLSIIDKEYNSGLGWKFLFTMKQNEMFLFPSEDFNPKENDLFDEKNLSLISKNMFRVQKFGELSKSGFWFRHHLETSVELKKELRSTSYLDFYSKDFMKTIVKVRLNHLGKIVQIGEY

SEQ ID NO: 90 - protein, 1453 aa, Sporocytophaga myxococcoides
MKTVLGLDLGTNSIGWALIQHDFDSKKGEILGMGSRIIPMSQDILGEFGKGNSVSQTADRTKFRSARRLRERHLLRRERLHRVLNILGFLPRHYAADIDFEKRLGQFFEGKEPKLAYDNNQFIFTKSFGKMLADFRQHQPDFLKDEKSNDLLIPYDWSIYYLRKEALTKKIEKEELAWIILNFNQKRGYYQLRGEEEEENLNKLVEFHSLKIIDVVADEKLNNKGETWYSLLLENGWTYRRSSKVPLFDWKEKVRDFIVTTDINDDGSVKTDKEGNEKRSFRAPSDDDWTLLKKKTEQDIDKSRKPIGAYIYDAILKNPKQKINGKLVRTVERKFYKEELKLILQKQKEFHPELQSTDLYNECIRELYKNNDAHQLQLNKKDFVHLFLEDIIFYQRPLRSQKSSVGNCPLEFRKFKDSEGIEKVEYLKTIPKSNPYFQEFRIWQWMYNLSIYKKDDDENVTRDFLKTIEDWEDLFEFLNHRKDIEQETLLKFLLGKNGVKGKALKVEAGKFRWNYVSDKIYPCNETKALIISKLEKVKGVEEKFLTEEIEYKLWHLIYSVTDKVEYEKALKAFAGKQKLDLVSFVDSFKRFPPFKNEYGAYSEKAIKKILPLLRTGKSWNWMAIDSKVRDRINKIITGEFDEEIKNKVREKAEKHSLKKENDFQGLPLWLAQYVVYGRHSEASFSGKWNSVDDLKKYLEEFKQHSLRNPIVEQVLTETLRVVADIWQFYGKGEKDFFSEIHIELGREMKNTAEDRKEMSAIIQANETTNLRIKALLNELLQDKKVENVRPYSPSQQEILKIYEDGVLSSDIEIPDDIQKISKAAQPTKSELQRYKLWLEQKYRSPYTGAMIPLGKLFTSEYEIEHIIPQSLYFDDSFSNKVICESAVNKLKDSRLGMEFIKECHGMVVETGFGKSVTVFEEETYRDFVVQNYSKNHSKKSKLLLEEIPEKMIERQMNDTRYISKFISSVLSNIVREEVNDDGVNSKNIVPGNGKITTQLKQDWGLNDIWNELILPRFERLNVLTDSKHFTAWSENHQRLLPTVPIGLSKGFSKKRIDHRHHALDALVIACASRNHINFLNNAHAIDKKKNSEEKQKFRHDLKAILCDKKYSDKSEKNYRWIFKKPWDNFTIDSKNALDKIIVSFKQNLRIINKATNRYEKWVDRDGIKVKEWHKQEGINWATRKPLHKDTVSGKVDLKRVTVPEGKILTATRKSLDTSFDLKVIESITDTGIQKILKNYLTSKSNNPELAFSSEGVEDMNKNIRKYNDGKLHQPIYKVRIFELGSKFPLGQFGNKKFKYVETAKGTNLFFAVYEDENKNRNYETIPLNVVIERQKQGLSSVPIKSEKGHKLLFYLSPNDIVYVPGSNEEFSIDRLYRFTDSSDKTANFIPLSVSSLIFSSNKNEQKKIGISYPIQDEFGLGSPQSKNQKSIDGIMIKEKCVKVNIDRLGRVSF

SEQ ID NO: 91 - protein, 1509 aa, Psychroflexus torquis
MKRILGLDLGTNSIGWSLIEHDFKNKQGQIEGLGVRIIPMSQEILGKFDAGQSISQTADRTKYRGVRRLYQRDNLRRERLHRVLKILDFLPKHYSESIDFQDKVGQFKPKQEVKLNYRKNEKNKHEFVFMNSFIEMVSEFKNAQPELFYNKGNGEETKIPYDWTLYYLRKKALTQQITKEELAWLILNFNQKRGYYQLRGEDIDEDKNKKYMQLKVNNLIDSGAKVKGKVLYNVIFDNGWKYEKQIVNKDEWEGRTKEFIITTKTLKNGNIKRTYKAVDSEIDWAAIKAKTEQDINKANKTVGEYIYESLLDNPSQKIRGKLVKTIERKFYKEEFEKLLSKQIELQPELFNESLYKACIKELYPRNENHQSNNKKQGFEYLFTEDIIFYQRPLKSQKSNISGCQFEHKIYKQKNKKTGKLELIKEPIKTISRSHPLFQEFRIWQWLQNLKIYNKEKIENGKLEDVTTQLLPNNEAYVTLFDFLNTKKELEQKQFIEYFVKKKLIDKKEKEHFRWNFVEDKKYPFSETRAQFLSRLAKVKGIKNTEDFLNKNTQVGSKENSPFIKRIEQLWHIIYSVSDLKEYEKALEKFAEKHNLEKDSFLKNFKKFPPFVSDYASYSKKAISKLLPIMRMGKYWSESAVPTQVKERSLSIMERVKVLPLKEGYSDKDLADLLSRVSDDDIPKQLIKSFISFKDKNPLKGLNTYQANYLVYGRHSETGDIQHWKTPEDIDRYLNNFKQHSLRNPIVEQVVMETLRVVRDIWEHYGNNEKDFFKEIHVELGREMKSPAGKREKLSQRNTENENTNHRIREVLKELMNDASVEGGVRDYSPSQQEILKLYEEGIYQNPNTNYLKVDEDEILKIRKKNNPTQKEIQRYKLWLEQGYISPYTGKIIPLTKLFTHEYQIEHIIPQSRYYDNSLGNKIICESEVNEDKDNKTAYEYLKVEKGSIVFGHKLLNLDEYEAHVNKYFKKNKTKLKNLLSEDIPEGFINRQLNDSRYISKLVKGLLSNIVRENGEQEATSKNLIPVTGVVTSKLKQDWGLNDKWNEIIAPRFKRLNKLTNSNDFGFWDNDINAFRIQVPDSLIKGFSKKRIDHRHHALDALVVACTSRNHTHYLSALNAENKNYSLRDKLVIKNENGDYTKTFQIPWQGFTIEAKNNLEKTVVSFKKNLRVINKTNNKFWSYKDENGNLNLGKDGKPKKKLRKQTKGYNWAIRKPLHKETVSGIYNINAPKNKIATSVRTLLTEIKNEKHLAKITDLRIRETILPNHLKHYLNNKGEANFSEAFSQGGIEDLNKKITTLNEGKKHQPIYRVKIFEVGSKFSISEDENSAKSKKYVEAAKGTNLFFAIYLDEENKKRNYETIPLNEVITHQKQVAGFPKSERLSVQPDSQKGTFLFTLSPNDLVYVPNNEELENRDLFNLGNLNVEQISRIYKFTDSSDKTCNFIPFQVSKLIFNLKKKEQKKLDVDFIIQNEFGLGSPQSKNQKSIDDVMIKEKCIKLKIDRLGNISKA

SEQ ID NO: 92 - DNA, 36 bp, Lactobacillus reuteri
gttttagatgtacttcaaatcaataatgtttagaac

SEQ ID NO: 93 - DNA, 36 bp, Lactobacillus rossiae
gttttagatgtatgtcagatcaatagggttaagaac

SEQ ID NO: 94 - DNA, 36 bp, Pediococcus pentosaceus
gtttcagaagagtgttaaatcaataagttcaagtac

SEQ ID NO: 95 - DNA, 36 bp, Lactobacillus nodensis
gttttagtactctcaagaatttagtaacagtaaaac

SEQ ID NO: 96 - DNA, 37 bp, Artificial sequence
  sequence from Sulfurospirillum sp. SCADC (Sspe)
acgacactttacaacaccatcgcttagcaactgraac

SEQ ID NO: 97 - DNA, 36 bp, Bifidobacterium thermophilum
caagtctatcaagaaggaaggatgctaattctcagc

SEQ ID NO: 98 - DNA, 36 bp, Loktanella vestfoldensis
attatagctgttcaaaattcgcggtccagccgcaac

SEQ ID NO: 99 - DNA, 36 bp, Sphingomonas sanxanigenens
accatagctgttcagagatcgcggtccagcggcaac

SEQ ID NO: 100 - DNA, 47 bp, Epilithonimonas tenax DSM
gttgttgtgtatcccaaagatacttaaaaatgaaagcaattcacaac

SEQ ID NO: 101 - DNA, 47 bp, Sporocytophaga myxococcoides
gttgtgatttgctttcaaacaacgatctttgaattatcggaaacaac

SEQ ID NO: 102 - DNA, 46 bp, Psychroflexus torquis
cctgtgaattatcactaaaaatacaattttgaaagcaattcacaac

SEQ ID NO: 103 - DNA, 36 bp, Lactobacillus reuteri
tttaactctgtacttcaaatcaataatatttagtag

SEQ ID NO: 104 - DNA, 37 bp, Lactobacillus rossiae
tttaacgctgtatgtcagatcaatagggtcaaaagtt

SEQ ID NO: 105 - DNA, 37 bp, Pediococcus pentosaceus
tttcaaaacagaatgttaaatcaataagtttaagtac

SEQ ID NO: 106 - DNA, 38 bp, Lactobacillus nodensis
gttttactgttactaaattcttgagaacctactaaaat

SEQ ID NO: 107 - DNA, 39 bp, artificial sequence
  sequence from Sulfurospirillum sp. SCADC (Sspe)
atttcagtgcatcgaacgatacgtgttgtaaagtgtcgt

SEQ ID NO: 108 - DNA, 36 bp, Bifidobacterium thermophilum
gtgtagcgcgatatactaaaaaagctaattctcagt

SEQ ID NO: 109 - DNA, 36 bp, Loktanella vestfoldensis
ttaacggctcgaccgcgaattttgaacatttggata

SEQ ID NO: 110 - DNA, 36 bp, Sphingomonas sanxanigenens
ttaaccgccagaccacgatctctgaagtgctcaggc

SEQ ID NO: 111 - DNA, 47 bp, Epilithonimonas tenax
attgtgaattgctttcggatacaaatgtagaaattaattatttatat

SEQ ID NO: 112 - DNA, 47 bp, Sporocytophaga myxococcoides
attgtgatttgctttcactagcaaatatatataaatttaattttatt

SEQ ID NO: 113 - DNA, 46 bp, Psychroflexus torquis
attgtgaattgcttcaaaattgtgtaccaaatatattaatattata

SEQ ID NO: 114 - RNA, 169 nt, Artificial Sequence
  synthesized Lreu Single Guide RNA
gggcgcuaaagaggaagaggacaguuuuagauguacuucgaaagaaguacagaguuaaaaucaaacaagugcuucagcacaaguuucuacuuuugagucaguuaucugaccaauacauaaaagggaauuaaaucguucacaugagcguuuuaauucccuuucucucuuu

SEQ ID NO: 115 - RNA, 166 nt, Artificial Sequence
  synthesized  Lros  Single Guide RNA
gggcgcuaaagaggaagaggacaguuuuagauguaugucgaaagacauacagcguuaaaaucaagcaaggcuuucgagccaaguuuaaaucuuuggguucgcuauucggaccguacauaguaaaagggcgucaucgaguucaaauucgauggcgcccuuuaguuuu

SEQ ID NO: 116 - RNA, 168 nt, Artificial Sequence
  synthesized  Ppen  Single Guide RN
gggcgcuaaagaggaagaggacaguuucagaagaguguugaaaaacauucuguuuugaaaucaaacaacgcuuuacgcggaguuuacacaucugucccauuauaugggcauuacauaauaaaagagaaaucaccuuuaagguugauuccucuuuuucuugcguuccuu

SEQ ID NO: 117 - RNA, 114 nt, Artificial Sequence2
  synthesized  Lnod Single Guide RNA
gggcgcuaaagaggaagaggacaguuuuaguacucucaaggaaacuugagaaccuacuaaaauaaggauuuauuccgaauuuaccaccuauuuuuuaauaggugguuuuuuuuu

SEQ ID NO: 118 - RNA, 180 nt, Artificial Sequence
  synthesized  Sspe  Single Guide RNA
gggcgcuaaagaggaagaggacaacgacacuuuacaacacgaaaguguuguaaagugucgugagugaaaguauagcauuuuucucaaaauaucgcacuuuuuuugcaaggaaauaauuugcgaaaaaaagagacaauuucgauacaagaaagccccaucaagucgaugauuuguaaggcu

SEQ ID NO: 119 - RNA, 117 nt, Artificial Sequence
  synthesized  Sspe Single Guide RNA (tracrRNA Antisense-crRNA Antisens
gggcgcuaaagaggaagaggacaguuccaguugcuaagcgaaaguucgaugcacugaaaucaucgaaaagauauauagacccgcccaacugccuuaggcauggcgggcuucuuucuu

SEQ ID NO: 120 - RNA, 254 nt, Artificial Sequence
  synthesized  Bthe  Single Guide RNA
gggcgcuaaagaggaagaggacagcugagaauuagcaucgaaaaaagcuaauucucaguaaguacagcaauuuauagcuguaucugaaugcuaagcgguuagccgcaggggagagcuucggcucuccccguucuuuucuagucgcacgugacacgccauagguagauugccugugagcaacucgagaauaguaguauucuucucuguaaaacgagacaucguugcugaugacuccauugacaaagaagggaauu

SEQ ID NO: 121 - RNA, 200 nt, Artificial Sequence
  synthesized Lves  Single Guide RNA
gggcgcuaaagaggaagaggacaguugcggcuggaccgcgaaagcggucgagccguuaacaagcauucgauugcaccacauugaaacgcaggcuacggccugcguuuucuuauuuccgguaugguucgucuugucaaagugucucagagaugcccgcuuucuaaauguggauugucgagguucgcacccguagcguuuuu

SEQ ID NO: 122 - RNA, 195 nt, Artificial Sequence
  synthesized  Ssan  Single Guide RNA
gggcgcuaaagaggaagaggacaguugccgcuggaccgcgaaaguggucuggcgguuaacaagcagccagucugcaccagauaagggcggcgcuccggcgccgccuuuuuuguuugcccggaauguugagacaggcgccaaaccauccccccuccccucggggcgugcggcaaucgcugcuuucagcucacucca

SEQ ID NO: 123 - RNA, 155 nt, Artificial Sequence
  synthesized  Eten Single Guide RNA
gggcgcuaaagaggaagaggacaguugugaauugcuuucgaaagaaagcaauucacaauaaggauuauuccguugugaaaacauuuagcaccucgccuaucugcgggguauuuuuuauuuaauacauucaaacaaugaagucgauugcauuuauu

SEQ ID NO: 124 - RNA, 149 nt, Artificial Sequences
  synthesized  Smyx Single Guide RNA
gggcgcuaaagaggaagaggacaguugugauuugcuuucgaaaaaagcaaaucacaauaaggauuauuccguugugaaaacauauaagccgccucgucuuacaauacggggcuuuuuuuauuccccauucacauauggccauccauuuu

SEQ ID NO: 125 - RNA, 155 nt, Artificial Sequence
  synthesized  Ptor Single Guide RNA
gggcgcuaaagaggaagaggacaguugugaauugcuuucagaaaugaagcaauucacaauaaggauuauuccguugugaaaacauuuaaagcggccuuuacgggucgcuuucuuuuuuuaaagaacuuaaacuuaauaaauucuuuacaaacuca

SEQ ID NO: 126 - DNA, 57 bp, Artificial sequence
  synthesized  GG-939
gactagacctgcaggggatcccgtcgacaaattctaaacgctaaagaggaagaggac

SEQ ID NO: 127 - RNA, 174 nt, Artificial sequence
  synthesized single guide RNA
  misc_feature (1)..(20): n is a, c, g, or u
nnnnnnnnnnnnnnnnnnnngcuauaguuccuuacugaaagguaaguugcuauaguaagggcaacagacccgaggcguuggggaucgccuagcccguuuuuacgggcucuccccauauucaaaauaaugacagacgagcaccuuggagcauuuauuuccgaggugcuuuuuuuu

SEQ ID NO: 128 - RNA, 166 nt, Artificial Sequence
  synthesized Lreu Single Guide RNA
  misc_feature (1)..(20): n is a, c, g, or u
nnnnnnnnnnnnnnnnnnnnguuuuagauguacuucgaaagaaguacagaguuaaaaucaaacaagugcuucagcacaaguuucuacuuuugagucaguuaucugaccaauacauaaaagggaauuaaaucguucacaugagcguuuuaauucccuuucucucuuu

SEQ ID NO: 129 - RNA, 163 nt, Artificial Sequence
  synthesized Lros Single Guide RNA
  misc_feature (1)..(20): n is a, c, g, or u
nnnnnnnnnnnnnnnnnnnnguuuuagauguaugucgaaagacauacagcguuaaaaucaagcaaggcuuucgagccaaguuuaaaucuuuggguucgcuauucggaccguacauaguaaaagggcgucaucgaguucaaauucgauggcgcccuuuaguuuu

SEQ ID NO: 130 - RNA, 165 nt, Artificial Sequence
  synthesized Ppen  Single Guide RNA
  misc_feature (1)..(20): n is a, c, g, or u
nnnnnnnnnnnnnnnnnnnnguuucagaagaguguugaaaaacauucuguuuugaaaucaaacaacgcuuuacgcggaguuuacacaucugucccauuauaugggcauuacauaauaaaagagaaaucaccuuuaagguugauuccucuuuuucuugcguuccuu

SEQ ID NO: 131 - RNA, 111 nt, Artificial Sequence
  synthesized  Lnod Single Guide RNA
  misc_feature (1)..(20): n is a, c, g, or u
nnnnnnnnnnnnnnnnnnnnguuuuaguacucucaaggaaacuugagaaccuacuaaaauaaggauuuauuccgaauuuaccaccuauuuuuuaauaggugguuuuuuuuu

SEQ ID NO: 132 - RNA, 177 nt, Artificial Sequence
  synthesized  Sspe  Single Guide RNA
  misc_feature (1)..(20): n is a, c, g, or u
nnnnnnnnnnnnnnnnnnnnacgacacuuuacaacacgaaaguguuguaaagugucgugagugaaaguauagcauuuuucucaaaauaucgcacuuuuuuugcaaggaaauaauuugcgaaaaaaagagacaauuucgauacaagaaagccccaucaagucgaugauuuguaaggcu

SEQ ID NO: 133 - RNA, 114 nt, Artificial Sequence
  synthesized  Sspe Single Guide RNA (tracrRNA Antisense-crRNA Antisense
  misc_feature (1)..(20): n is a, c, g, or u
nnnnnnnnnnnnnnnnnnnnguuccaguugcuaagcgaaaguucgaugcacugaaaucaucgaaaagauauauagacccgcccaacugccuuaggcauggcgggcuucuuucuu

SEQ ID NO: 134 - RNA, 251 nt, Artificial Sequence
  synthesized  Bthe  Single Guide RNA
  misc_feature (1)..(20): n is a, c, g, or u
nnnnnnnnnnnnnnnnnnnngcugagaauuagcaucgaaaaaagcuaauucucaguaaguacagcaauuuauagcuguaucugaaugcuaagcgguuagccgcaggggagagcuucggcucuccccguucuuuucuagucgcacgugacacgccauagguagauugccugugagcaacucgagaauaguaguauucuucucuguaaaacgagacaucguugcugaugacuccauugacaaagaagggaauu

SEQ ID NO: 135 - RNA, 197 nt, Artificial Sequence
  synthesized  Lves  Single Guide RNA
  misc_feature (1)..(20): n is a, c, g, or u
nnnnnnnnnnnnnnnnnnnnguugcggcuggaccgcgaaagcggucgagccguuaacaagcauucgauugcaccacauugaaacgcaggcuacggccugcguuuucuuauuuccgguaugguucgucuugucaaagugucucagagaugcccgcuuucuaaauguggauugucgagguucgcacccguagcguuuuu

SEQ ID NO: 136 - RNA, 192 nt, Artificial Sequence
  synthesized  Ssan Single Guide RNA
  misc_feature (1)..(20): n is a, c, g, or u
nnnnnnnnnnnnnnnnnnnnguugccgcuggaccgcgaaaguggucuggcgguuaacaagcagccagucugcaccagauaagggcggcgcuccggcgccgccuuuuuuguuugcccggaauguugagacaggcgccaaaccauccccccuccccucggggcgugcggcaaucgcugcuuucagcucacucca

SEQ ID NO: 137 - RNA, 152 nt, Artificial Sequence
  synthesized  Eten  Single Guide RNA
  misc_feature (1)..(20): n is a, c, g, or u
nnnnnnnnnnnnnnnnnnnnguugugaauugcuuucgaaagaaagcaauucacaauaaggauuauuccguugugaaaacauuuagcaccucgccuaucugcgggguauuuuuuauuuaauacauucaaacaaugaagucgauugcauuuauu

SEQ ID NO: 138 - RNA, 146 nt, Artificial Sequence
  synthesized  Smyx  Single Guide RNA
  misc_feature (1)..(20): n is a, c, g, or u
nnnnnnnnnnnnnnnnnnnnguugugauuugcuuucgaaaaaagcaaaucacaauaaggauuauuccguugugaaaacauauaagccgccucgucuuacaauacggggcuuuuuuuauuccccauucacauauggccauccauuuu

SEQ ID NO: 139 - RNA, 152 nt, Artificial Sequence
  synthesized  Ptor  Single Guide RNA
  misc_feature (1)..(20): n is a, c, g, or u
nnnnnnnnnnnnnnnnnnnnguugugaauugcuuucagaaaugaagcaauucacaauaaggauuauuccguugugaaaacauuuaaagcggccuuuacgggucgcuuucuuuuuuuaaagaacuuaaacuuaauaaauucuuuacaaacuca

SEQ ID NO: 140 - protein, 1092 aa, Brevibacillus laterosporus
MAYTMGIDVGIASCGWAIVDLERQRIIDIGVRTFEKAENPKNGEALAVPRREARSSRRRLRRKKHRIERLKHMFVRNGLAVDIQHLEQTLRSQNEIDVWQLRVDGLDRMLTQKEWLRVLIHLAQRRGFQSNRKTDGSSEDGQVLVNVTENDRLMEEKDYRTVAEMMVKDEKFSDHKRNKNGNYHGVVSRSSLLVEIHTLFETQRQHHNSLASKDFELEYVNIWSAQRPVATKDQIEKMIGTCTFLPKEKRAPKASWHFQYFMLLQTINHIRITNVQGTRSLNKEEIEQVVNMALTKSKVSYHDTRKILDLSEEYQFVGLDYGKEDEKKKVESKETIIKLDDYHKLNKIFNEVELAKGETWEADDYDTVAYALTFFKDDEDIRDYLQNKYKDSKNRLVKNLANKEYTNELIGKVSTLSFRKVGHLSLKALRKIIPFLEQGMTYDKACQAAGFDFQGISKKKRSVVLPVIDQISNPVVNRALTQTRKVINALIKKYGSPETIHIETARELSKTFDERKNITKDYKENRDKNEHAKKHLSELGIINPTGLDIVKYKLWCEQQGRCMYSNQPISFERLKESGYTEVDHIIPYSRSMNDSYNNRVLVMTRENREKGNQTPFEYMGNDTQRWYEFEQRVTTNPQIKKEKRQNLLLKGFTNRRELEMLERNLNDTRYITKYLSHFISTNLEFSPSDKKKKVVNTSGRITSHLRSRWGLEKNRGQNDLHHAMDAIVIAVTSDSFIQQVTNYYKRKERRELNGDDKFPLPWKFFREEVIARLSPNPKEQIEALPNHFYSEDELADLQPIFVSRMPKRSITGEAHQAQFRRVVGKTKEGKNITAKKTALVDISYDKNGDFNMYGRETDPATYEAIKERYLEFGGNVKKAFSTDLHKPKKDGTKGPLIKSVRIMENKTLVHPVNKGKGVVYNSSIVRTDVFQRKEKYYLLPVYVTDVTKGKLPNKVIVAKKGYHDWIEVDDSFTFLFSLYPNDLIFIRQNPKKKISLKKRIESHSISDSKEVQEIHAYYKGVDSSTAAIEFIIHDGSYYAKGVGVQNLDCFEKYQVDILGNYFKVKGEKRLELETSDSNHKGKDVNSIKSTSR

SEQ ID NO: 141 - RNA, 20 nt, Artificial Sequence
  synthesized  Variable Targeting domain T1
cgcuaaagaggaagaggaca

SEQ ID NO: 142 - RNA, 20 nt, Artificial Sequence
  synthesized  Variable Targeting domain T2-5
ucuagauagauuacgaauuc

SEQ ID NO: 143 - RNA, 20 nt, Artificial Sequence
  synthesized  Variable Targeting domain T2-7
ccggcgacguugggucaacu

SEQ ID NO: 144 - RNA, 105 nt, Artificial Sequence
  synthesized  Spy sgRNA T2
gggucuagauagauuacgaauucguuuuagagcuagaaauagcaaguuaaaauaaggcuaguccguuaucaacuugaaaaaguggcaccgagucggugcuuuuuu

SEQ ID NO: 145 - RNA, 123 nt, Artificial Sequence
  synthesized  Sth3 sgRNA T2
gggucuagauagauuacgaauucguuuuagagcuguguuguuucgguuaaaacaacacagcgaguuaaaauaaggcuuaguccguacucaacuugaaaagguggcaccgauucgguguuuuuu

SEQ ID NO: 146 - RNA, 122 nt, Artificial Sequence
  synthesized  Sth1 sgRNA T1
gggcgcuaaagaggaagaggacaguuuuuguacucucaagauucaauaaucuugcagaagcuacaaagauaaggcuucaugccgaaaucaacacccugucauuuuauggcaggguguuuucg

SEQ ID NO: 147 - RNA, 122 nt, Artificial Sequence
  synthesized  Sth1 sgRNA T2
gggccggcgacguugggucaacuguuuuuguacucucaagauucaauaaucuugcagaagcuacaaagauaaggcuucaugccgaaaucaacacccugucauuuuauggcaggguguuuucg

SEQ ID NO: 148 - RNA, 20 nt, Artificial Sequence
  synthesized  shifted T1 variable targeting domain, T1-3
aaacgcuaaagaggaagagg

SEQ ID NO: 149 - RNA, 177 nt, Artificial Sequence
  synthesized  Blat sgRNA (T1)-3
gggaaacgcuaaagaggaagagggcuauaguuccuuacugaaagguaaguugcuauaguaagggcaacagacccgaggcguuggggaucgccuagcccguuuuuacgggcucuccccauauucaaaauaaugacagacgagcaccuuggagcauuuauuuccgaggugcuuuuuuuu

SEQ ID NO: 150 - protein, 9 aa, Simian virus
MAPKKKRKV

SEQ ID NO: 151 - protein, 18 aa, Agrobacterium tumefaciens
KRPRDRHDGELGGRKRAR

SEQ ID NO: 152 - RNA, 147 nt, Brevibacillus laterosporus
gcuauaguuccuuacugaaagguaaguugcuauaguaagggcaacagacccgaggcguuggggaucgccuagcccguuuuuacgggcucuccccauauucaaaauaaugacagacgagcaccuuggagcauuuauuuccgaggugcu

SEQ ID NO: 153 - RNA, 147 nt, Brevibacillus laterosporus
gcuauaguuccuuacugaaagguaaguugcuauaguaagggcaacagacccgaggcguuggggaucgccuagcccguguuuacgggcucuccccauauucaaaauaaugacagacgagcaccuuggagcauuuaucuccgaggugcu

SEQ ID NO: 154 - DNA, 73 bp, Zea mays
ccttgaccaggataatgaggtactggctggaaggcccaagagcgggcgaggtagaggtgttcgcgaacctgcc

SEQ ID NO: 155 - DNA, 73 bp, Zea mays
cttgaccaggataatgaggtactggcttggaaggcccaagagcgggcgaggtagaggtgttcgcgaacctgcc

SEQ ID NO: 156 - DNA, 73 bp, Zea mays
cttgaccaggataatgaggtactggctaggaaggcccaagagcgggcgaggtagaggtgttcgcgaacctgcc

SEQ ID NO: 157 - DNA, 73 bp, Zea mays
cttgaccaggataatgaggtactggctgggaaggcccaagagcgggcgaggtagaggtgttcgcgaacctgcc

SEQ ID NO: 158 - DNA, 73 bp, Zea mays
cttgaccaggataatgaggtactggctcggaaggcccaagagcgggcgaggtagaggtgttcgcgaacctgcc

SEQ ID NO: 159 - DNA, 72 bp, Zea mays
ccttgaccaggataatgaggtactggcggaaggcccaagagcgggcgaggtagaggtgttcgcgaacctgcc

SEQ ID NO: 160 - DNA, 73 bp, Zea mays
ttgaccaggataatgaggtactggctttggaaggcccaagagcgggcgaggtagaggtgttcgcgaacctgcc

SEQ ID NO: 161 - DNA, 73 bp, Zea mays
cttgaccaggataatgaggtactggcgtggaaggcccaagagcgggcgaggtagaggtgttcgcgaacctgcc

SEQ ID NO: 162 - DNA, 71 bp, Zea mays
ccttgaccaggataatgaggtactggctaaggcccaagagcgggcgaggtagaggtgttcgcgaacctgcc

SEQ ID NO: 163 - DNA, 42 bp, Zea mays
ccttgaccaggataatgaggtagaggtgttcgcgaacctgcc

SEQ ID NO: 164 - DNA, 65 bp, Zea mays
ccttgaccaggataatgaggtactggcccaagagcgggcgaggtagaggtgttcgcgaacctgcc

SEQ ID NO: 165 - DNA, 73 bp, Zea mays; identical to SEQ ID NO: 155

SEQ ID NO: 166 - DNA, 72 bp, Zea mays; identical to SEQ ID NO: 159

SEQ ID NO: 167 - DNA, 69 bp, Zea mays
ccttgaccaggataatgaggtactggaaggcccaagagcgggcgaggtagaggtgttcgcgaacctgcc

SEQ ID NO: 168 - DNA, 72 bp, Zea mays
ccttgaccaggataatgaggtactggtggaaggcccaagagcgggcgaggtagaggtgttcgcgaacctgcc

SEQ ID NO: 169 - DNA, 73 bp, Zea mays; identical to SEQ ID NO: 161

SEQ ID NO: 170 - DNA, 53 bp, Zea mays
ccttgaccaggataatgaggtactggcgaggtagaggtgttcgcgaacctgcc

SEQ ID NO: 171 - DNA, 42 bp, Zea mays; identical to SEQ ID NO: 163

SEQ ID NO: 172 - DNA, 68 bp, Zea mays
ccttgaccaggataatgaggtacggaaggcccaagagcgggcgaggtagaggtgttcgcgaacctgcc

SEQ ID NO: 173 - DNA, 73 bp, Zea mays; identical to SEQ ID NO: 156

SEQ ID NO: 174 - DNA, 67 bp, Zea mays
ccttgaccaggataatgaggtaggaaggcccaagagcgggcgaggtagaggtgttcgcgaacctgcc

SEQ ID NO: 175 - DNA, 28 bp, Artificial Sequence
  synthesized sequence TK-113
gaaattctaaacgctaaagaggaagagg

SEQ ID NO: 176 - DNA, 60 bp, Artificial Sequence
  synthesized sequence JKYS921.1
ctacactctttccctacacgacgctcttccgatctggaataaacgctaaagaggaagagg

SEQ ID NO: 177 - DNA, 43 bp, Artificial Sequence; identical to SEQ ID NO: 8
  synthesized sequence JKY557

SEQ ID NO: 178 - DNA, 18 bp, Artificial Sequence
  synthesized sequence  JKY558
caagcagaagacggcata

SEQ ID NO: 179 - DNA, 21 bp, Artificial Sequence
  synthesized sequence pUC-EheD
ccgcatcaggcgccattcgcc

SEQ ID NO: 180 - DNA, 22 bp, Artificial Sequence
  synthesized sequence pUC-LguR
gcgaggaagcggaagagcgccc

SEQ ID NO: 181 - DNA, 58 bp, Artificial Sequence
  synthesized sequence JKYX1.1
ctacactctttccctacacgacgctcttccgatctaaggggcgctggccctcctagtc

SEQ ID NO: 182 - DNA, 54 bp, Artificial Sequence
  synthesized sequence JKYS178Rd
caagcagaagacggcatacgagctcttccgatctgccggctggcattgtctctg

SEQ ID NO: 183 - DNA, 58 bp, Artificial Sequence
  synthesized sequence JKYS1083.1
ctacactctttccctacacgacgctcttccgatctggaaggcaggttcgcgaacacct

SEQ ID NO: 184 - DNA, 57 bp, Artificial Sequence
  synthesized sequence JKYS1084
caagcagaagacggcatacgagctcttccgatctctccgagacaacaaactgcaggt

SEQ ID NO: 185 - DNA, 55 bp, Artificial Sequence
  synthesized sequence  JKYX2.1
ctacactctttccctacacgacgctcttccgatctaaggggccggacgcggtgtt

SEQ ID NO: 186 - DNA, 58 bp, Artificial Sequence
  synthesized sequence JKYX3
caagcagaagacggcatacgagctcttccgatcttacatgcgcaggtgcaaagtctac

SEQ ID NO: 187 - DNA, 22 bp, Artificial Sequence
  synthesized sequence in Figure 40
agaggaagaggacagtcccgaa

SEQ ID NO: 188 - DNA, 12 bp, Artificial Sequence
  synthesized sequence in Figure 40
  misc_feature (1)..(1): n is a, c, g, or t
ntgtcagggctt

SEQ ID NO: 189 - DNA, 22 bp, Artificial Sequence
  synthesized sequence in Figure 40
tctccttctcctgtcagggctt

SEQ ID NO: 190 - DNA, 12 bp, Artificial Sequence
  synthesized sequence in Figure 40
  misc_feature (12)..(12): n is a, c, g, or t
agaggaagaggn

SEQ ID NO: 191 - DNA, 28 bp, Artificial Sequence
  synthesized sequence in Figure 40
cgctaaagaggaagaggacagtcccgaa

SEQ ID NO: 192 - DNA, 28 bp, Artificial Sequence
  synthesized sequence in Figure 40
gcgatttctccttctcctgtcagggctt

SEQ ID NO: 193 - RNA, 20 nt, Artificial sequence
  synthesized Variable Targeting domain-direct
cgcuaaagaggaagaggaca

SEQ ID NO: 194 - RNA, 20 nt, Artificial sequence
  symthesized Variable Targeting domain-reverse
cgcuaaagaggaagaggaca

SEQ ID NO: 195 - RNA, 16 nt, Brevibacillus laterosporus
gcuauaguuccuuacu

SEQ ID NO: 196 - RNA, 16 nt, Brevibacillus laterosporus
aucauaucauaucgag

SEQ ID NO: 197 - RNA, 16 nt, Brevibacillus laterosporus
gguaaguugcuauagu

SEQ ID NO: 198 - RNA, 16 nt, Brevibacillus laterosporus
cuugauaugauaugau

SEQ ID NO: 199 - RNA, 118 nt, Brevibacillus laterosporus; identical to SEQ ID NO: 68

SEQ ID NO: 200 - RNA, 59 nt, Brevibacillus laterosporus
acuuucauuuuauauccauauaucaucgaagucaaucucauuuaucugucuauuuuaug

SEQ ID NO: 201 - RNA, 16 nt, Lactobacillus reuteri
guuuuagauguacuuc

SEQ ID NO: 202 - RNA, 16 nt, Lactobacillus rossiae
guuuuagauguauguc

SEQ ID NO: 203 - RNA, 16 nt, Pediococcus pentosaceus
guuucagaagaguguu

SEQ ID NO: 204 - RNA, 17 nt, Lactobacillus nodensis
guuuuaguacucucaag

SEQ ID NO: 205 - RNA, 17 nt, Artificial Sequence
  sequence from Sulfurospirillum species SCADC (Sspe)
acgacacuuuacaacac

SEQ ID NO: 206 - RNA, 16 nt, Artificial Sequence
  sequence from Sulfurospirillum species SCADC (Sspe)
guuccaguugcuaagc

SEQ ID NO: 207 - RNA, 16 nt, Bifidobacterium thermophilum
gcugagaauuagcauc

SEQ ID NO: 208 - RNA, 16 nt, Loktanella vestfoldensis
guugcggcuggaccgc

SEQ ID NO: 209 - RNA, 16 nt, Sphingomonas sanxanigenens
guugccgcuggaccgc

SEQ ID NO: 210 - RNA, 16 nt, Epilithonimonas tenax
guugugaauugcuuuc

SEQ ID NO: 211 - RNA, 16 nt, Sporocytophaga myxococcoides
guugugauuugcuuuc

SEQ ID NO: 212 - RNA, 17 nt, Psychroflexus torquis
guugugaauugcuuuca

SEQ ID NO: 213 - RNA, 18 nt, Lactobacillus reuteri
gaaguacagaguuaaaau

SEQ ID NO: 214 - RNA, 18 nt, Lactobacillus rossiae
gacauacagcguuaaaau

SEQ ID NO: 215 - RNA, 18 nt, Pediococcus pentosaceus
aacauucuguuuugaaau

SEQ ID NO: 216 - RNA, 19 nt, Lactobacillus nodensis
cuugagaaccuacuaaaau

SEQ ID NO: 217 - RNA, 17 nt, Artificial Sequence
  sequence from Sulfurospirillum species SCADC (Sspe)
guguuguaaagugucgu

SEQ ID NO: 218 - RNA, 13 nt, Artificial Sequence
  sequence from Sulfurospirillum species SCADC (Sspe)
guucgaugcacug

SEQ ID NO: 219 - RNA, 16 nt, Bifidobacterium thermophilum
aaagcuaauucucagu

SEQ ID NO: 220 - RNA, 17 nt, Loktanella vestfoldensis
gcggucgagccguuaac

SEQ ID NO: 221 - RNA, 17 nt, Sphingomonas sanxanigenens
guggucuggcgguuaac

SEQ ID NO: 222 - RNA, 16 nt, Epilithonimonas tenax
gaaagcaauucacaau

SEQ ID NO: 223 - RNA, 15 nt, Sporocytophaga myxococcoides
aaagcaaaucacaau

SEQ ID NO: 224 - RNA, 16 nt, Psychroflexus torquis
ugaagcaauucacaau

SEQ ID NO: 225 - RNA, 108 nt, Lactobacillus reuteri
caaacaagugcuucagcacaaguuucuacuuuugagucaguuaucugaccaauacauaaaagggaauuaaaucguucacaugagcguuuuaauucccuuucucucuuu

SEQ ID NO: 226 - RNA, 105 nt, Lactobacillus rossiae
caagcaaggcuuucgagccaaguuuaaaucuuuggguucgcuauucggaccguacauaguaaaagggcgucaucgaguucaaauucgauggcgcccuuuaguuuu

SEQ ID NO: 227 - RNA, 107 nt, Pediococcus pentosaceus
caaacaacgcuuuacgcggaguuuacacaucugucccauuauaugggcauuacauaauaaaagagaaaucaccuuuaagguugauuccucuuuuucuugcguuccuu

SEQ ID NO: 228 - RNA, 51 nt, Lactobacillus nodensis
aaggauuuauuccgaauuuaccaccuauuuuuuaauaggugguuuuuuuuu

SEQ ID NO: 229 - RNA, 119 nt, Artificial Sequence
  sequence from Sulfurospirillum species SCADC (Sspe)
gagugaaaguauagcauuuuucucaaaauaucgcacuuuuuuugcaaggaaauaauuugcgaaaaaaagagacaauuucgauacaagaaagccccaucaagucgaugauuuguaaggcu

SEQ ID NO: 230 - RNA, 61 nt, Artificial Sequence
  sequence from Sulfurospirillum species SCADC (Sspe)
aaaucaucgaaaagauauauagacccgcccaacugccuuaggcauggcgggcuucuuucuu

SEQ ID NO: 231 - RNA, 195 nt, Bifidobacterium thermophilum
aaguacagcaauuuauagcuguaucugaaugcuaagcgguuagccgcaggggagagcuucggcucuccccguucuuuucuagucgcacgugacacgccauagguagauugccugugagcaacucgagaauaguaguauucuucucuguaaaacgagacaucguugcugaugacuccauugacaaagaagggaauu

SEQ ID NO: 232 - RNA, 140 nt, Loktanella vestfoldensis
aagcauucgauugcaccacauugaaacgcaggcuacggccugcguuuucuuauuuccgguaugguucgucuugucaaagugucucagagaugcccgcuuucuaaauguggauugucgagguucgcacccguagcguuuuu

SEQ ID NO: 233 - RNA, 135 nt, Sphingomonas sanxanigenens
aagcagccagucugcaccagauaagggcggcgcuccggcgccgccuuuuuuguuugcccggaauguugagacaggcgccaaaccauccccccuccccucggggcgugcggcaaucgcugcuuucagcucacucca

SEQ ID NO: 234 - RNA, 96 nt, Epilithonimonas tenax
aaggauuauuccguugugaaaacauuuagcaccucgccuaucugcgggguauuuuuuauuuaauacauucaaacaaugaagucgauugcauuuauu

SEQ ID NO: 235 - RNA, 91 nt, Sporocytophaga myxococcoides
aaggauuauuccguugugaaaacauauaagccgccucgucuuacaauacggggcuuuuuuuauuccccauucacauauggccauccauuuu

SEQ ID NO: 236 - RNA, 95 nt, Psychroflexus torquis
aaggauuauuccguugugaaaacauuuaaagcggccuuuacgggucgcuuucuuuuuuuaaagaacuuaaacuuaauaaauucuuuacaaacuca